European Patent Application EP 4 260 871 A1, published October 18, 2023. Title: Optic neuro protective agent comprising anti-LRP1 antibody. Applicant: Tokyo University of Pharmacy and Life Sciences National institutes of biomedical innovation, health and nutrition. The sequence listing filed with the application follows.

SEQUENCE LISTING (25 sequences)

SEQ ID NO: 1 - protein, 4544 aa, Homo sapiens
MLTPPLLLLLPLLSALVAAAIDAPKTCSPKQFACRDQITCISKGWRCDGERDCPDGSDEAPEICPQSKAQRCQPNEHNCLGTELCVPMSRLCNGVQDCMDGSDEGPHCRELQGNCSRLGCQHHCVPTLDGPTCYCNSSFQLQADGKTCKDFDECSVYGTCSQLCTNTDGSFICGCVEGYLLQPDNRSCKAKNEPVDRPPVLLIANSQNILATYLSGAQVSTITPTSTRQTTAMDFSYANETVCWVHVGDSAAQTQLKCARMPGLKGFVDEHTINISLSLHHVEQMAIDWLTGNFYFVDDIDDRIFVCNRNGDTCVTLLDLELYNPKGIALDPAMGKVFFTDYGQIPKVERCDMDGQNRTKLVDSKIVFPHGITLDLVSRLVYWADAYLDYIEVVDYEGKGRQTIIQGILIEHLYGLTVFENYLYATNSDNANAQQKTSVIRVNRFNSTEYQVVTRVDKGGALHIYHQRRQPRVRSHACENDQYGKPGGCSDICLLANSHKARTCRCRSGFSLGSDGKSCKKPEHELFLVYGKGRPGIIRGMDMGAKVPDEHMIPIENLMNPRALDFHAETGFIYFADTTSYLIGRQKIDGTERETILKDGIHNVEGVAVDWMGDNLYWTDDGPKKTISVARLEKAAQTRKTLIEGKMTHPRAIVVDPLNGWMYWTDWEEDPKDSRRGRLERAWMDGSHRDIFVTSKTVLWPNGLSLDIPAGRLYWVDAFYDRIETILLNGTDRKIVYEGPELNHAFGLCHHGNYLFWTEYRSGSVYRLERGVGGAPPTVTLLRSERPPIFEIRMYDAQQQQVGTNKCRVNNGGCSSLCLATPGSRQCACAEDQVLDADGVTCLANPSYVPPPQCQPGEFACANSRCIQERWKCDGDNDCLDNSDEAPALCHQHTCPSDRFKCENNRCIPNRWLCDGDNDCGNSEDESNATCSARTCPPNQFSCASGRCIPISWTCDLDDDCGDRSDESASCAYPTCFPLTQFTCNNGRCININWRCDNDNDCGDNSDEAGCSHSCSSTQFKCNSGRCIPEHWTCDGDNDCGDYSDETHANCTNQATRPPGGCHTDEFQCRLDGLCIPLRWRCDGDTDCMDSSDEKSCEGVTHVCDPSVKFGCKDSARCISKAWVCDGDNDCEDNSDEENCESLACRPPSHPCANNTSVCLPPDKLCDGNDDCGDGSDEGELCDQCSLNNGGCSHNCSVAPGEGIVCSCPLGMELGPDNHTCQIQSYCAKHLKCSQKCDQNKFSVKCSCYEGWVLEPDGESCRSLDPFKPFIIFSNRHEIRRIDLHKGDYSVLVPGLRNTIALDFHLSQSALYWTDVVEDKIYRGKLLDNGALTSFEVVIQYGLATPEGLAVDWIAGNIYWVESNLDQIEVAKLDGTLRTTLLAGDIEHPRAIALDPRDGILFWTDWDASLPRIEAASMSGAGRRTVHRETGSGGWPNGLTVDYLEKRILWIDARSDAIYSARYDGSGHMEVLRGHEFLSHPFAVTLYGGEVYWTDWRTNTLAKANKWTGHNVTVVQRTNTQPFDLQVYHPSRQPMAPNPCEANGGQGPCSHLCLINYNRTVSCACPHLMKLHKDNTTCYEFKKFLLYARQMEIRGVDLDAPYYNYIISFTVPDIDNVTVLDYDAREQRVYWSDVRTQAIKRAFINGTGVETVVSADLPNAHGLAVDWVSRNLFWTSYDTNKKQINVARLDGSFKNAVVQGLEQPHGLVVHPLRGKLYWTDGDNISMANMDGSNRTLLFSGQKGPVGLAIDFPESKLYWISSGNHTINRCNLDGSGLEVIDAMRSQLGKATALAIMGDKLWWADQVSEKMGTCSKADGSGSVVLRNSTTLVMHMKVYDESIQLDHKGTNPCSVNNGDCSQLCLPTSETTRSCMCTAGYSLRSGQQACEGVGSFLLYSVHEGIRGIPLDPNDKSDALVPVSGTSLAVGIDFHAENDTIYWVDMGLSTISRAKRDQTWREDVVTNGIGRVEGIAVDWIAGNIYWTDQGFDVIEVARLNGSFRYVVISQGLDKPRAITVHPEKGYLFWTEWGQYPRIERSRLDGTERVVLVNVSISWPNGISVDYQDGKLYWCDARTDKIERIDLETGENREVVLSSNNMDMFSVSVFEDFIYWSDRTHANGSIKRGSKDNATDSVPLRTGIGVQLKDIKVFNRDRQKGTNVCAVANGGCQQLCLYRGRGQRACACAHGMLAEDGASCREYAGYLLYSERTILKSIHLSDERNLNAPVQPFEDPEHMKNVIALAFDYRAGTSPGTPNRIFFSDIHFGNIQQINDDGSRRITIVENVGSVEGLAYHRGWDTLYWTSYTTSTITRHTVDQTRPGAFERETVITMSGDDHPRAFVLDECQNLMFWTNWNEQHPSIMRAALSGANVLTLIEKDIRTPNGLAIDHRAEKLYFSDATLDKIERCEYDGSHRYVILKSEPVHPFGLAVYGEHIFWTDWVRRAVQRANKHVGSNMKLLRVDIPQQPMGIIAVANDTNSCELSPCRINNGGCQDLCLLTHQGHVNCSCRGGRILQDDLTCRAVNSSCRAQDEFECANGECINFSLTCDGVPHCKDKSDEKPSYCNSRRCKKTFRQCSNGRCVSNMLWCNGADDCGDGSDEIPCNKTACGVGEFRCRDGTCIGNSSRCNQFVDCEDASDEMNCSATDCSSYFRLGVKGVLFQPCERTSLCYAPSWVCDGANDCGDYSDERDCPGVKRPRCPLNYFACPSGRCIPMSWTCDKEDDCEHGEDETHCNKFCSEAQFECQNHRCISKQWLCDGSDDCGDGSDEAAHCEGKTCGPSSFSCPGTHVCVPERWLCDGDKDCADGADESIAAGCLYNSTCDDREFMCQNRQCIPKHFVCDHDRDCADGSDESPECEYPTCGPSEFRCANGRCLSSRQWECDGENDCHDQSDEAPKNPHCTSQEHKCNASSQFLCSSGRCVAEALLCNGQDDCGDSSDERGCHINECLSRKLSGCSQDCEDLKIGFKCRCRPGFRLKDDGRTCADVDECSTTFPCSQRCINTHGSYKCLCVEGYAPRGGDPHSCKAVTDEEPFLIFANRYYLRKLNLDGSNYTLLKQGLNNAVALDFDYREQMIYWTDVTTQGSMIRRMHLNGSNVQVLHRTGLSNPDGLAVDWVGGNLYWCDKGRDTIEVSKLNGAYRTVLVSSGLREPRALVVDVQNGYLYWTDWGDHSLIGRIGMDGSSRSVIVDTKITWPNGLTLDYVTERIYWADAREDYIEFASLDGSNRHVVLSQDIPHIFALTLFEDYVYWTDWETKSINRAHKTTGTNKTLLISTLHRPMDLHVFHALRQPDVPNHPCKVNNGGCSNLCLLSPGGGHKCACPTNFYLGSDGRTCVSNCTASQFVCKNDKCIPFWWKCDTEDDCGDHSDEPPDCPEFKCRPGQFQCSTGICTNPAFICDGDNDCQDNSDEANCDIHVCLPSQFKCTNTNRCIPGIFRCNGQDNCGDGEDERDCPEVTCAPNQFQCSITKRCIPRVWVCDRDNDCVDGSDEPANCTQMTCGVDEFRCKDSGRCIPARWKCDGEDDCGDGSDEPKEECDERTCEPYQFRCKNNRCVPGRWQCDYDNDCGDNSDEESCTPRPCSESEFSCANGRCIAGRWKCDGDHDCADGSDEKDCTPRCDMDQFQCKSGHCIPLRWRCDADADCMDGSDEEACGTGVRTCPLDEFQCNNTLCKPLAWKCDGEDDCGDNSDENPEECARFVCPPNRPFRCKNDRVCLWIGRQCDGTDNCGDGTDEEDCEPPTAHTTHCKDKKEFLCRNQRCLSSSLRCNMFDDCGDGSDEEDCSIDPKLTSCATNASICGDEARCVRTEKAAYCACRSGFHTVPGQPGCQDINECLRFGTCSQLCNNTKGGHLCSCARNFMKTHNTCKAEGSEYQVLYIADDNEIRSLFPGHPHSAYEQAFQGDESVRIDAMDVHVKAGRVYWTNWHTGTISYRSLPPAAPPTTSNRHRRQIDRGVTHLNISGLKMPRGIAIDWVAGNVYWTDSGRDVIEVAQMKGENRKTLISGMIDEPHAIVVDPLRGTMYWSDWGNHPKIETAAMDGTLRETLVQDNIQWPTGLAVDYHNERLYWADAKLSVIGSIRLNGTDPIVAADSKRGLSHPFSIDVFEDYIYGVTYINNRVFKIHKFGHSPLVNLTGGLSHASDVVLYHQHKQPEVTNPCDRKKCEWLCLLSPSGPVCTCPNGKRLDNGTCVPVPSPTPPPDAPRPGTCNLQCFNGGSCFLNARRQPKCRCQPRYTGDKCELDQCWEHCRNGGTCAASPSGMPTCRCPTGFTGPKCTQQVCAGYCANNSTCTVNQGNQPQCRCLPGFLGDRCQYRQCSGYCENFGTCQMAADGSRQCRCTAYFEGSRCEVNKCSRCLEGACVVNKQSGDVTCNCTDGRVAPSCLTCVGHCSNGGSCTMNSKMMPECQCPPHMTGPRCEEHVFSQQQPGHIASILIPLLLLLLLVLVAGVVFWYKRRVQGAKGFQHQRMTNGAMNVEIGNPTYKMYEGGEPDDVGGLLDADFALDPDKPTNFTNPVYATLYMGGHGSRHSLASTDEKRELLGRGPEDEIGDPLA

SEQ ID NO: 2 - protein, 4545 aa, Mus musculus
MLTPPLLLLLPLLSALVSGATMDAPKTCSPKQFACRDQITCISKGWRCDGERDCPDGSDEAPEICPQSKAQRCPPNEHSCLGTELCVPMSRLCNGIQDCMDGSDEGAHCRELRANCSRMGCQHHCVPTPSGPTCYCNSSFQLQADGKTCKDFDECSVYGTCSQLCTNTDGSFTCGCVEGYLLQPDNRSCKAKNEPVDRPPVLLIANSQNILATYLSGAQVSTITPTSTRQTTAMDFSYANETVCWVHVGDSAAQTQLKCARMPGLKGFVDEHTINISLSLHHVEQMAIDWLTGNFYFVDDIDDRIFVCNRNGDTCVTLLDLELYNPKGIALDPAMGKVFFTDYGQIPKVERCDMDGQNRTKLVDSKIVFPHGITLDLVSRLVYWADAYLDYIEVVDYEGKGRQTIIQGILIEHLYGLTVFENYLYATNSDNANTQQKTSVIRVNRFNSTEYQVVTRVDKGGALHIYHQRRQPRVRSHACENDQYGKPGGCSDICLLANSHKARTCRCRSGFSLGSDGKSCKKPEHELFLVYGKGRPGIIRGMDMGAKVPDEHMIPIENLMNPRALDFHAETGFIYFADTTSYLIGRQKIDGTERETILKDGIHNVEGVAVDWMGDNLYWTDDGPKKTISVARLEKAAQTRKTLIEGKMTHPRAIVVDPLNGWMYWTDWEEDPKDSRRGRLERAWMDGSHRDIFVTSKTVLWPNGLSLDIPAGRLYWVDAFYDRIETILLNGTDRKIVYEGPELNHAFGLCHHGNYLFWTEYRSGSVYRLERGVAGAPPTVTLLRSERPPIFEIRMYDAQQQQVGTNKCRVNNGGCSSLCLATPGSRQCACAEDQVLDTDGVTCLANPSYVPPPQCQPGEFACANNRCIQERWKCDGDNDCLDNSDEAPALCHQHTCPSDRFKCENNRCIPNRWLCDGDNDCGNSEDESNATCSARTCPPNQFSCASGRCIPISWTCDLDDDCGDRSDESASCAYPTCFPLTQFTCNNGRCININWRCDNDNDCGDNSDEAGCSHSCSSTQFKCNSGRCIPEHWTCDGDNDCGDYSDETHANCTNQATRPPGGCHSDEFQCRLDGLCIPLRWRCDGDTDCMDSSDEKSCEGVTHVCDPNVKFGCKDSARCISKAWVCDGDSDCEDNSDEENCEALACRPPSHPCANNTSVCLPPDKLCDGKDDCGDGSDEGELCDQCSLNNGGCSHNCSVAPGEGIVCSCPLGMELGSDNHTCQIQSYCAKHLKCSQKCDQNKFSVKCSCYEGWVLEPDGESCRSLDPFKPFIIFSNRHEIRRIDLHKGDYSVLVPGLRNTIALDFHLSQSALYWTDVVEDKIYRGKLLDNGALTSFEVVIQYGLATPEGLAVDWIAGNIYWVESNLDQIEVAKLDGTLRTTLLAGDIEHPRAIALDPRDGILFWTDWDASLPRIEAASMSGAGRRTIHRETGSGGWPNGLTVDYLEKRILWIDARSDAIYSARYDGSGHMEVLRGHEFLSHPFAVTLYGGEVYWTDWRTNTLAKANKWTGHNVTVVQRTNTQPFDLQVYHPSRQPMAPNPCEANGGRGPCSHLCLINYNRTVSCACPHLMKLHKDNTTCYEFKKFLLYARQMEIRGVDLDAPYYNYIISFTVPDIDNVTVLDYDAREQRVYWSDVRTQAIKRAFINGTGVETVVSADLPNAHGLAVDWVSRNLFWTSYDTNKKQINVARLDGSFKNAVVQGLEQPHGLVVHPLRGKLYWTDGDNISMANMDGSNHTLLFSGQKGPVGLAIDFPESKLYWISSGNHTINRCNLDGSELEVIDTMRSQLGKATALAIMGDKLWWADQVSEKMGTCNKADGSGSVVLRNSTTLVMHMKVYDESIQLEHEGTNPCSVNNGDCSQLCLPTSETTRSCMCTAGYSLRSGQQACEGVGSFLLYSVHEGIRGIPLDPNDKSDALVPVSGTSLAVGIDFHAENDTIYWVDMGLSTISRAKRDQTWREDVVTNGIGRVEGIAVDWIAGNIYWTDQGFDVIEVARLNGSFRYVVISQGLDKPRAITVHPEKGYLFWTEWGHYPRIERSRLDGTERVVLVNVSISWPNGISVDYQGGKLYWCDARMDKIERIDLETGENREVVLSSNNMDMFSVSVFEDFIYWSDRTHANGSIKRGCKDNATDSVPLRTGIGVQLKDIKVFNRDRQKGTNVCAVANGGCQQLCLYRGGGQRACACAHGMLAEDGASCREYAGYLLYSERTILKSIHLSDERNLNAPVQPFEDPEHMKNVIALAFDYRAGTSPGTPNRIFFSDIHFGNIQQINDDGSGRTTIVENVGSVEGLAYHRGWDTLYWTSYTTSTITRHTVDQTRPGAFERETVITMSGDDHPRAFVLDECQNLMFWTNWNELHPSIMRAALSGANVLTLIEKDIRTPNGLAIDHRAEKLYFSDATLDKIERCEYDGSHRYVILKSEPVHPFGLAVYGEHIFWTDWVRRAVQRANKYVGSDMKLLRVDIPQQPMGIIAVANDTNSCELSPCRINNGGCQDLCLLTHQGHVNCSCRGGRILQEDFTCRAVNSSCRAQDEFECANGECISFSLTCDGVSHCKDKSDEKPSYCNSRRCKKTFRQCNNGRCVSNMLWCNGVDDCGDGSDEIPCNKTACGVGEFRCRDGSCIGNSSRCNQFVDCEDASDEMNCSTTDCSSYFRLGVKGVLFQPCERTSLCYAPSWVCDGANDCGDYSDERDCPGVKRPRCPLNYFACPSGRCIPMSWTCDKEDDCENGEDETHCNKFCSEAQFECQNHRCISKQWLCDGSDDCGDGSDEAAHCEGKTCGPSSFSCPGTHVCVPERWLCDGDKDCTDGADESVTAGCLYNSTCDDREFMCQNRLCIPKHFVCDHDRDCADGSDESPECEYPTCGPNEFRCANGRCLSSRQWECDGENDCHDHSDEAPKNPHCTSPEHKCNASSQFLCSSGRCVAEALLCNGQDDCGDGSDERGCHVNECLSRKLSGCSQDCEDLKIGFKCRCRPGFRLKDDGRTCADLDECSTTFPCSQLCINTHGSYKCLCVEGYAPRGGDPHSCKAVTDEEPFLIFANRYYLRKLNLDGSNYTLLKQGLNNAVALDFDYREQMIYWTDVTTQGSMIRRMHLNGSNVQVLHRTGLSNPDGLAVDWVGGNLYWCDKGRDTIEVSKLNGAYRTVLVSSGLREPRALVVDVQNGYLYWTDWGDHSLIGRIGMDGSGRSIIVDTKITWPNGLTVDYVTERIYWADAREDYIEFASLDGSNRHVVLSQDIPHIFALTLFEDYVYWTDWETKSINRAHKTTGANKTLLISTLHRPMDLHVFHALRQPDVPNHPCKVNNGGCSNLCLLSPGGGHKCACPTNFYLGGDGRTCVSNCTASQFVCKNDKCIPFWWKCDTEDDCGDHSDEPPDCPEFKCRPGQFQCSTGICTNPAFICDGDNDCQDNSDEANCDIHVCLPSQFKCTNTNRCIPGIFRCNGQDNCGDGEDERDCPEVTCAPNQFQCSITKRCIPRVWVCDRDNDCVDGSDEPANCTQMTCGVDEFRCKDSGRCIPARWKCDGEDDCGDGSDEPKEECDERTCEPYQFRCKNNRCVPGRWQCDYDNDCGDNSDEESCTPRPCSESEFSCANGRCIAGRWKCDGDHDCADGSDEKDCTPRCDMDQFQCKSGHCIPLRWRCDADADCMDGSDEEACGTGVRTCPLDEFQCNNTLCKPLAWKCDGEDDCGDNSDENPEECARFICPPNRPFRCKNDRVCLWIGRQCDGVDNCGDGTDEEDCEPPTAQNPHCKDKKEFLCRNQRCLSSSLRCNMFDDCGDGSDEEDCSIDPKLTSCATNASMCGDEARCVRTEKAAYCACRSGFHTVPGQPGCQDINECLRFGTCSQLCNNTKGGHLCSCARNFMKTHNTCKAEGSEYQVLYIADDNEIRSLFPGHPHSAYEQTFQGDESVRIDAMDVHVKAGRVYWTNWHTGTISYRSLPPAAPPTTSNRHRRQIDRGVTHLNISGLKMPRGIAIDWVAGNVYWTDSGRDVIEVAQMKGENRKTLISGMIDEPHAIVVDPLRGTMYWSDWGNHPKIETAAMDGTLRETLVQDNIQWPTGLAVDYHNERLYWADAKLSVIGSIRLNGTDPIVAADSKRGLSHPFSIDVFEDYIYGVTYINNRVFKIHKFGHSPLINLTGGLSHASDVVLYHQHKQPEVTNPCDRKKCEWLCLLSPSGPVCTCPNGKRLDNGTCVPVPSPTPPPDAPRPGTCTLQCFNGGSCFLNARRQPKCRCQPRYTGDKCELDQCWEYCHNGGTCAASPSGMPTCRCPTGFTGPKCTAQVCAGYCSNNSTCTVNQGNQPQCRCLPGFLGDRCQYRQCSGFCENFGTCQMAADGSRQCRCTVYFEGPRCEVNKCSRCLQGACVVNKQTGDVTCNCTDGRVAPSCLTCIDHCSNGGSCTMNSKMMPECQCPPHMTGPRCEEQVVSQQQPGHMASILIPLLLLLLLLLVAGVVFWYKRRVRGAKGFQHQRMTNGAMNVEIGNPTYKMYEGGEPDDVGGLLDADFALDPDKPTNFTNPVYATLYMGGHGSRHSLASTDEKRELLGRGPEDEIGDPLA

SEQ ID NO: 3 - protein, 4544 aa, Macaca mulatta
MLTPPLLLLLPLLSALVAAAIDAPKTCSPKQFACRDQITCISKGWRCDGERDCPDGSDEAPEICPQSKAQRCQPNEHNCLGTELCVPMSRLCNGVQDCMDGSDEGPHCRELRGNCSRLGCQHHCVPTLDGPTCYCNSSFQLQADSKTCKDFDECSVYGTCSQLCTNTDGSFICGCVEGYLLQPDNRSCKAKNEPVDRPPVLLIANSQNILATYLSGAQVSTITPTSTRQTTAMDFSYANETVCWVHVGDNAAQTQLKCARMPGLKGFVDEHTINISLSLHHVEQMAIDWLTGNFYFVDDIDDRIFVCNRNGDTCVTLLDLELYNPKGIALDPAMGKVFFTDYGQIPKVERCDMDGQNRTKLVDSKIVFPHGITLDLVSRLVYWADAYLDYIEVVDYEGKGRQTIIQGILIEHLYGLTVFENYLYATNSDNANAQQKTSVIRVNRFNSTEYQVVTRVDKGGALHIYHQRRQPRVRSHACENDQYGKPGGCSDICLLANSHKARTCRCRSGFSLGSDGKSCKKPEHELFLVYGKGRPGIIRGMDMGAKVPDEHMIPIENLMNPRALDFHAETGFIYFADTTSYLIGRQKIDGTERETILKDGIHNVEGVAVDWMGDNLYWTDDGPKKTISVARLEKAAQTRKTLIEGKMTHPRAIVVDPLNGWMYWTDWEEDPKDSRRGRLERAWMDGSHRDIFVTSKTVLWPNGLSLDIPAGRLYWVDAFYDRIETILLNGTDRKIVYEGPELNHAFGLCHHGNYLFWTEYRSGSVYRLERGVGGAPPTVTLLRSERPPIFEIRMYDAQQQQVGTNKCRVNNGGCSSLCLATPGSRQCACAEDQVLDADGVTCLANPSYVPPPQCQPGEFACANSRCIQERWKCDGDNDCLDNSDEAPALCHQHTCPSDRFKCENNRCIPNRWLCDGDNDCGNSEDESNATCSARTCPPNQFSCASGRCIPISWTCDLDDDCGDRSDESASCAYPTCFPLTQFTCNNGRCININWRCDNDNDCGDNSDEAGCSHSCSSTQFKCNSGRCIPEHWTCDGDNDCGDYSDETHANCTNQATRPPGGCHTDEFQCRLDGLCIPLRWRCDGDTDCMDSSDEKSCEGVTHVCDPSVKFGCKDSARCISKAWVCDGDNDCEDNSDEENCESLACRPPSHPCANNTSVCLPPDKLCDGNDDCGDGSDEGELCDQCSLNNGGCSHNCSVAPGEGIVCSCPLGMELGPDNHTCQIQSYCAKHLKCSQKCDQNKFSVKCSCYEGWVLEPDGESCRSLDPFKPFIIFSNRHEIRRIDLHKGDYSVLVPGLRNTIALDFHLSQSALYWTDVVEDKIYRGKLLDNGALTSFEVVIQYGLATPEGLAVDWIAGNIYWVESNLDQIEVAKLDGTLRTTLLAGDIEHPRAIALDPRDGILFWTDWDASLPRIEAASMSGAGRRTVHRETGSGGWPNGLTVDYLEKRILWIDARSDAIYSARYDGSGHMEVLRGHEFLSHPFAVTLYGGEVYWTDWRTNTLAKANKWTGHNVTVVQRTNTQPFDLQVYHPSRQPMAPNPCEANGGRGPCSHLCLINYNRTVSCACPHLMKLHKDKTTCYEFKKFLLYARQMEIRGVDLDAPYYNYIISFTVPDIDNVTVLDYDAREQRVYWSDVRTQAIKRAFINGTGVETVVSADLPNAHGLAVDWVSRNLFWTSYDTNKKQINVARLDGSFKNAVVQGLEQPHGLVVHPLRGKLYWTDGDNISMANMDGSNRTLLFSGQKGPVGLAIDFPESKLYWISSGNHTINRCNLDGSGLEVIDAMRSQLGKATALAIMGDKLWWADQVSEKMGTCSKADGSGSIVLRNSTTLVMHMKVYDESIQLDHKGTNPCSVNNGDCSQLCLPTSETTRSCMCTAGYSLRSGQQACEGVGSFLLYSVHEGIRGIPLDPNDKSDALVPVSGTSLAVGIDFHAENDTIYWVDMGLSTISRAKRDQTWREDVVTNGIGRVEGIAVDWIAGNIYWTDQGFDVIEVARLNGSFRYVVISQGLDKPRAITVHPEKGYLFWTEWGQYPRIERSRLDGTERVVLVNVSISWPNGISVDYQDGKLYWCDARTDKIERIDLETGENREVVLSSNNMDMFSVSVFEDFIYWSDRTHANGSIKRGSKDNATDSVPLRTGIGVQLKDIKVFNRDRQKGTNVCAVANGGCQQLCLYRGRGQRACACAHGMLAEDGASCREYAGYLLYSERTILKSIHLSDERNLNAPVQPFEDPEHMKNVIALAFDYRAGTSPGTPNRIFFSDIHFGNIQQINDDGSRRITIVENVGSVEGLAYHRGWDTLYWTSYTTSTITRHTVDQTRPGAFERETVITMSGDDHPRAFVLDECQNLMFWTNWNEQHPSIMRAALSGANVLTLIEKDIRTPNGLAIDHRAEKLYFSDATLDKIERCEYDGSHRYVILKSEPVHPFGLAVYGEHIFWTDWVRRAVQRANKHVGSNMKLLRVDIPQQPMGIIAVANDTNSCELSPCRINNGGCQDLCLLTHQGHVNCSCRGGRILQDDLTCRAVNSSCRAQDEFECANGECINFSLTCDGVPHCKDKSDEKPSYCNSRRCKKTFRQCSNGRCVSNMLWCNGADDCGDGSDEIPCNKTACGVGEFRCRDGTCIGNSSRCNQFVDCEDASDEMNCSATDCSSYFRLGVKGVLFQPCERTSLCYAPSWVCDGANDCGDYSDERDCPGVKRPRCPLNYFACPSGRCIPMSWTCDKEDDCEHGEDETHCNKFCSEAQFECQNHRCISKQWLCDGSDDCGDGSDEAAHCEGKTCGPSSFSCPGTHVCVPERWLCDGDKDCADGADESIAAGCLYNSTCDDREFMCQNRQCIPKHFVCDHDRDCADGSDESPECEYPTCGPSEFRCANGRCLSSRQWECDGENDCHDQSDEAPKNPHCTSPEHKCNASSQFLCSSGRCVAEVLLCNGQDDCGDGSDERGCHINECLSHKLSGCSQDCEDLKIGFKCRCRPGFRLKDDGRTCADVDECSTTFPCSQRCINTHGSYKCLCVEGYAPRGGDPHSCKAVTDEEPFLIFANRYYLRKLNLDGSNYTLLKQGLNNAVALDFDYREQMIYWTDVTTQGSMIRRMHLNGSNVQVLHRTGLSNPDGLAVDWVGGNLYWCDKGRDTIEVSKLNGAYRTVLVSSGLREPRALVVDVQNGYLYWTDWGDHSLIGRIGMDGSSRSVIVDTKITWPNGLTLDYVTERIYWADAREDYIEFASLDGSNRHVVLSQDIPHIFALTLFEDYVYWTDWETKSINRAHKTTGTNKTLLISTLHRPMDLHVFHALRQPDVPNHPCKVNNGGCSNLCLLSPGGGHKCACPTNFYLGSDGRTCVSNCTASQFVCKNDKCIPFWWKCDTEDDCGDHSDEPPDCPEFKCRPGQFQCSTGICTNPAFICDGDNDCQDNSDEANCDIHVCLPSQFKCTNTNRCIPGIFRCNGQDNCGDGEDERDCPEVTCAPNQFQCSITKRCIPRVWVCDRDNDCVDGSDEPANCTQMTCGVDEFRCKDSGRCIPARWKCDGEDDCGDGSDEPKEECDERTCEPYQFRCKNNRCVPGRWQCDYDNDCGDNSDEESCTPRPCSESEFSCANGRCIAGRWKCDGDHDCADGSDEKDCTPRCDMDQFQCKSGHCIPLRWRCDADADCMDGSDEEACGTGVRTCPLDEFQCNNTLCKPLAWKCDGEDDCGDNSDENPEECARFVCPPNRPFRCKNDRVCLWIGRQCDGMDNCGDGTDEEDCEPPTAQTTHCKDKKEFLCRNQRCLSSSLRCNMFDDCGDGSDEEDCSIDPKLTSCATNASICGDEARCVRTEKAAYCACRSGFHTVPGQPGCQDINECLRFGTCSQLCNNTKGGHLCSCARNFMKTHNTCKAEGSEYQVLYIADDNEIRSLFPGHPHSAYEQAFQGDESVRIDAMDVHVKAGRVYWTNWHTGTISYRSLPPAAPPTTSNRHRRQIDRGVTHLNISGLKMPRGIAIDWVAGNVYWTDSGRDVIEVAQMKGENRKTLISGMIDEPHAIVVDPLRGTMYWSDWGNHPKIETAAMDGTLRETLVQDNIQWPTGLAVDYHNERLYWADAKLSVIGSIRLNGTDPIVAADSKRGLSHPFSIDVFEDYIYGVTYINNRVFKIHKFGHSPLVNLTGGLSHASDVVLYHQHKQPEVTNPCDRKKCEWLCLLSPSGPVCTCPNGKRLDNGTCVPVPSPTPPPDAPRPGTCNLQCFNGGSCFLNARRQPKCRCQPRYTGDKCELDQCWEHCRNGGTCAASPSGMPTCRCPTGFTGPKCTQQVCAGYCANNSTCTVNQGNQPQCRCLPGFLGDRCQYRQCSGYCENFGTCQMAADGSRQCRCTAYFEGLRCEVNKCSRCLEGACVVNKQSGDVTCNCTDGRVAPSCLTCIGHCSNGGSCTMNSKMMPECQCPPHMTGPRCEEHVFSQQQPGHIASILIPLLLLLLVLLVAGVVFWYKRRVQGAKGFQHQRMTNGAMNVEIGNPTYKMYEGGEPDDVGGLLDADFALDPDKPTNFTNPVYATLYMGGHGSRHSLASTDEKRELLGRGPEDEIGDPLA

SEQ ID NO: 4 - protein, 4545 aa, Rattus norvegicus
MLTPPLLLLLPLLSALVAGATMDAPKTCSPKQFACRDQITCISKGWRCDGERDCPDGSDEAPEICPQSKAQRCPPNEHSCLGTELCVPMSRLCNGIQDCMDGSDEGAHCRELRVNCSRMGCQHHCVPTPSGPTCYCNNSFQLQADGKTCKDFDECSVYGTCSQLCTNTDGSFTCGCVEGYLLQPDNRSCKAKNEPVDRPPVLLIANSQNILATYLSGAQVSTITPTSTRQTTAMDFSYANETVCWVHVGDSAAQTQLKCARMPSLKGFVDEHTINISLSLHHVEQMAIDWLTGNFYFVDDIDDRIFVCNRNGDTCVTLLDLELYNPKGIALDPAMGKVFFTDYGQIPKVERCDMDGQNRTKLVDSKIVFPHGITLDLVSRLVYWADAYLDYIEVVDYEGKGRQTIIQGILIEHLYGLTVFENYLYATNSDNANTQQKTSVIRVNRFNSTEYQVVTRVDKGGALHIYHQRRQPRVRSHACENDQYGKPGGCSDICLLANSHKARTCRCRSGFSLGSDGKSCKKPEHELFLVYGKGRPGIIRGMDMGAKVPDEHMIPIENLMNPRALDFHAETGFIYFADTTSYLIGRQKIDGTERETILKDGIHNVEGVAVDWMGDNLYWTDDGPKKTISVARLEKAAQTRKTLIEGKMTHPRAIVVDPLNGWMYWTDWEEDPKDSRRGRLERAWMDGSHRDIFVTSKTVLWPNGLSLDIPAGRLYWVDAFYDRIETILLNGTDRKIVYEGPELNHAFGLCHHGNYLFWTEYRSGSVYRLERGVAGAQPTVTLLRSERPPIFEIRMYDAQQQQVGTNKCRVNNGGCSSLCLATPGSRQCACAEDQVLDADGVTCLANPSYVPPPQCQPGEFACANNRCIQERWKCDGDNDCLDNSDEAPALCHQHTCPSDRFKCENNRCIPNRWLCDGDNDCGNSEDESNATCSARTCPPNQFSCASGRCIPISWTCDLDDDCGDRSDESASCAYPTCFPLTQFTCNNGRCININWRCDNDNDCGDNSDEAGCSHSCSSTQFKCNSGRCIPEHWTCDGDNDCGDYSDETHANCTNQATRPPGGCHSDEFQCRLDGLCIPLRWRCDGDTDCMDSSDEKGCEGVTHVCDPNVKFGCKDSARCISKAWVCDGDSDCEDNSDEENCEALACRPPSHPCANNTSVCLSPDKLCDGKDDCGDGSDEGELCDQCSLNNGGCSHNCSVAPGEGIVCSCPLGMELGPDNHTCQIQSYCAKHLKCSQKCDQNKFSVKCSCYEGWVLEPDGESCRSLDPFKPFIIFSNRHEIRRIDLHKGDYSVLVPGLRNTIALDFHLSQSALYWTDVVEDKIYRGKLLDNGALTSFEVVIQYGLATPEGLAVDWIAGNIYWVESNLDQIEVAKLDGTLRTTLLAGDIEHPRAIALDPRDGILFWTDWDASLPRIEAASMSGAGRRTIHRETGSGGWPNGLTVDYLEKRILWIDARSDAIYSARYDGSGHMEVLRGHEFLSHPFAVTLYGGEVYWTDWRTNTLAKANKWTGHNVTVVQRTNTQPFDLQVYHPSRQPMAPNPCEANGGRGPCSHLCLINYNRTVSCACPHLMKLHNDNTTCYEFKKFLLYARQMEIRGVDLDAPYYNYIISFTVPDIDNVTVLDYDAREQRVYWSDVRTQAIKRAFINGTGVETVVSADLPNAHGLAVDWVSRNLFWTSYDTNKKQINVARLDGSFKNAVVQGLEQPHGLVVHPLRGKLYWTDGDNISMVNMDGSNRTLLFSGQKGPVGLAIDFPESKLYWISSGNHTINRCNLDGSELEVIDTMRSQLGKATALAIMGDKLWWADQVSEKMGTCNKADGSGSVVLRNSTTLVMHMKVYDESIQLEHEGTNPCSVNNGDCSQLCLPTSETTRSCMCTAGYSLRSGQQACEGVGSFLLYSVHEGIRGIPLDPNDKSDALVPVSGTSLAVGIDFHAENDTIYWVDMGLSTISRAKRDQTWREDVVTNGIGRVEGIAVDWIAGNIYWTDQGFDVIEVARLNGSFRYVVISQGLDKPRAITVHPEKGYLFWTEWGHYPRIERSRLDGTERVVLVNVSISWPNGISVDYQGGKLYWCDARMDKIERIDLETGENREVVLSSNNMDMFSVSVFEDFIYWSDRTHANGSIKRGCKDNATDSVPLRTGIGVQLKDIKVFNRDRQKGTNVCAVANGGCQQLCLYRGGGQRACACAHGMLAEDGASCREYAGYLLYSERTILKSIHLSDERNLNAPVQPFEDPEHMKNVIALAFDYRAGTSPGTPNRIFFSDIHFGNIQQINDDGSGRTTIVENVGSVEGLAYHRGWDTLYWTSYTTSTITRHTVDQTRPGAFERETVITMSGDDHPRAFVLDECQNLMFWTNWNELHPSIMRAALSGANVLTLIEKDIRTPNGLAIDHRAEKLYFSDATLDKIERCEYDGSHRYVILKSEPVHPFGLAVYGEHIFWTDWVRRAVQRANKYVGSDMKLLRVDIPQQPMGIIAVANDTNSCELSPCRINNGGCQDLCLLTHQGHVNCSCRGGRILQEDFTCRAMNSSCRAQDEFECANGECISFSLTCDGVSHCKDKSDEKPSYCNSRRCKKTFRQCNNGRCVSNMLWCNGVDDCGDGSDEIPCNKTACGVGEFRCRDGSCIGNSSRCNQFVDCEDASDEMNCSATDCSSYFRLGVKGVLFQPCERTSLCYAPSWVCDGANDCGDYSDERDCPGVKRPRCPLNYFACPSGRCIPMSWTCDKEDDCENGEDETHCNKFCSEAQFECQNHRCISKQWLCDGSDDCGDGSDEAAHCEGKTCGPSSFSCPGTHVCVPERWLCDGDKDCADGADESISAGCLYNSTCDDREFMCQNRLCIPKHFVCDHDRDCADGSDESPECEYPTCGPNEFRCANGRCLSSRQWECDGENDCHDHSDEAPKNPHCTSPEHKCNASSQFLCSSGRCVAEALLCNGQDDCGDGSDERGCHVNECLSRKLSGCSQDCEDLKIGFKCRCRPGFRLKDDGRTCADVDECSTTFPCSQLCINTHGSYKCLCVEGYAPRGGDPHSCKAVTDEEPFLIFANRYYLRKLNLDGSNYTLLKQGLNNAVALDFDYRGQMIYWTDVTTQGSMIRRMHLNGSNVQVLHRTGLSNPDGLAVDWVGGNLYWCDKGRDTIEVSKLNGAYRTVLVSSGLREPRALVVDVQNGYLYWTDWGDHSLIGRIGMDGSGRSIIVDTKITWPNGLTVDYVTERIYWADAREDYIEFASLDGSNRHVVLSQDIPHIFALTLFEDYVYWTDWETKSINRAHKTTGANKTLLISTLHRPMDLHVFHALRQPDVPNHPCKVNNGGCSNLCLLSPGGGHKCACPTNFYLGGDGRTCVSNCTASQFVCKNDKCIPFWWKCDTEDDCGDHSDEPPDCPEFKCRPGQFQCSTGICTNPAFICDGDNDCQDNSDEANCDIHVCLPSQFKCTNTNRCIPGIFRCNGQDNCGDGEDERDCPEVTCAPNQFQCSITKRCIPRVWVCDRDNDCVDGSDEPANCTQMTCGVDEFRCKDSGRCIPARWKCDGEDDCGDGSDEPKEECDERTCEPYQFRCKNNRCVPGRWQCDYDNDCGDNSDEESCTPRPCSESEFSCANGRCIAGRWKCDGDHDCADGSDEKDCTPRCDMDQFQCKSGHCIPLRWRCDADADCMDGSDEEACGTGVRTCPLDEFQCNNTLCKPLAWKCDGEDDCGDNSDENPEECTRFQCPPNRPFRCKNDRVCLWIGRQCDGTDNCGDGTDEEDCEPPTAQNPHCKDKKEFLCRNQRCLSSSLRCNMFDDCGDGSDEEDCSIDPKLTSCATNASMCGDEARCVRTEKAAYCACRPGFHTVPGQPGCQDINECLRFGTCSQLCNNTKGGHLCSCARNFMKTHNTCKAEGSEYQVLYIADDNEIRSLFPGHPHSAYEQAFQGDESVRIDAMDVHVKAGRVYWTNWHTGTISYRSLPPAAPPTTSNRHRRQIDRGVTHLNISGLKMPRGIAIDWVAGNVYWTDSGRDVIEVAQMKGENRKTLISGMIDEPHAIVVDPLRGTMYWSDWGNHPKIETAAMDGTLRETLVQDNIQWPTGLAVDYHNERLYWADAKLSVIGSIRLNGTDPIVAVDSKRGLSHPFSIDVFEDYIYGVTYINNRVFKIHKFGHSPLINLTGGLSHASDVVLYHQHKQPEVTNPCDRKKCEWLCLLSPSGPVCTCPNGKRLDNGTCVPVPSPTPPPDAPRPGTCTLQCFNGGSCFLNARRQPKCRCQPRYTGDKCELDQCWEYCHNGGTCAASPSGMPTCRCPTGFTGPRCTQQVCAGYCANNSTCTVNQGNQPQCRCLPGFLGDRCQYRQCSGFCENFGTCQMAADGSRQCRCTVYFEGTRCEVNKCSRCLQGACVVNKQTGDVTCNCTDGRVAPSCLTCIDHCSNGGSCTMNSKMMPECQCPPHMTGPRCEEQVVSQQQPGHMTSILIPLLLLLLLLLVAGVVFWYKRRVRGAKGFQHQRMTNGAMNVEIGNPTYKMYEGGEPDDVGGLLDADFALDPDKPTNFTNPVYATLYMGGHGSRHSLASTDEKRELLGRGPEDEIGDPLA

SEQ ID NO: 5 - DNA, 14923 bp, Homo sapiens
acttcagtccggggaacagcggtgcgagctccaggcccatgcactgaggaggcggaaacaaggggagcccccagagctccatcaagccccctccaaaggctcccctacccggtccacgccccccaccccccctccccgcctcctcccaattgtgcatttttgcagccggaggcggctccgagatggggctgtgagcttcgcccggggagggggaaagagcagcgaggagtgaagcgggggggtggggtgaagggtttggatttcggggcagggggcgcacccccgtcagcaggccctccccaaggggctcggaactctacctcttcacccacgcccctggtgcgctttgccgaaggaaagaataagaacagagaaggaggagggggaaaggaggaaaagggggaccccccaactggggggggtgaaggagagaagtagcaggaccagaggggaaggggctgctgcttgcatcagcccacaccatgctgaccccgccgttgctcctgctgctgcccctgctctcagctctggtcgcggcggctatcgacgcccctaagacttgcagccccaagcagtttgcctgcagagatcaaataacctgtatctcaaagggctggcggtgcgacggtgagagggactgcccagacggatctgacgaggcccctgagatttgtccacagagtaaggcccagcgatgccagccaaacgagcataactgcctgggtactgagctgtgtgttcccatgtcccgcctctgcaatggggtccaggactgcatggacggctcagatgaggggccccactgccgagagctccaaggcaactgctctcgcctgggctgccagcaccattgtgtccccacactcgatgggcccacctgctactgcaacagcagctttcagcttcaggcagatggcaagacctgcaaagattttgatgagtgctcagtgtacggcacctgcagccagctatgcaccaacacagacggctccttcatatgtggctgtgttgaaggatacctcctgcagccggataaccgctcctgcaaggccaagaacgagccagtagaccggccccctgtgctgttgatagccaactcccagaacatcttggccacgtacctgagtggggcccaggtgtctaccatcacacctacgagcacgcggcagaccacagccatggacttcagctatgccaacgagaccgtatgctgggtgcatgttggggacagtgctgctcagacgcagctcaagtgtgcccgcatgcctggcctaaagggcttcgtggatgagcacaccatcaacatctccctcagtctgcaccacgtggaacagatggccatcgactggctgacaggcaacttctactttgtggatgacatcgatgataggatctttgtctgcaacagaaatggggacacatgtgtcacattgctagacctggaactctacaaccccaagggcattgccctggaccctgccatggggaaggtgtttttcactgactatgggcagatcccaaaggtggaacgctgtgacatggatgggcagaaccgcaccaagctcgtcgacagcaagattgtgtttcctcatggcatcacgctggacctggtcagccgccttgtctactgggcagatgcctatctggactatattgaagtggtggactatgagggcaagggccgccagaccatcatccagggcatcctgattgagcacctgtacggcctgactgtgtttgagaattatctctatgccaccaactcggacaatgccaatgcccagcagaagacgagtgtgatccgtgtgaaccgctttaacagcaccgagtaccaggttgtcacccgggtggacaagggtggtgccctccacatctaccaccagaggcgtcagccccgagtgaggagccatgcctgtgaaaacgaccagtatgggaagccgggtggctgctctgacatctgcctgctggccaacagccacaaggcgcggacctgccgctgccgttccggcttcagcctgggcagtgacgggaagtcatgcaagaagccggagcatgagctgttcctcgtgtatggcaagggccggccaggcatcatccggggcatggatatgggggccaaggtcccggatgagcacatgatccccattgaaaacctcatgaacccccgagccctggacttccacgctgagaccggcttcatctactttgccgacaccaccagctacctcattggccgccagaagattgatggcactgagcgggagaccatcctgaaggacggcatccacaatgtggagggtgtggccgtggactggatgggagacaatctgtactggacggacgatgggcccaaaaagacaatcagcgtggccaggctggagaaagctgctcagacccgcaagactttaatcgagggcaaaatgacacaccccagggctattgtggtggatccactcaatgggtggatgtactggacagactgggaggaggaccccaaggacagtcggcgtgggcggctggagagggcgtggatggatggctcacaccgagacatctttgtcacctccaagacagtgctttggcccaatgggctaagcctggacatcccggctgggcgcctctactgggtggatgccttctacgaccgcatcgagacgatactgctcaatggcacagaccggaagattgtgtatgaaggtcctgagctgaaccacgcctttggcctgtgtcaccatggcaactacctcttctggactgagtatcggagtggcagtgtctaccgcttggaacggggtgtaggaggcgcaccccccactgtgacccttctgcgcagtgagcggccccccatctttgagatccgaatgtatgatgcccagcagcagcaagttggcaccaacaaatgccgggtgaacaatggcggctgcagcagcctgtgcttggccacccctgggagccgccagtgcgcctgtgctgaggaccaggtgttggacgcagacggcgtcacttgcttggcgaacccatcctacgtgcctccaccccagtgccagccaggcgagtttgcctgtgccaacagccgctgcatccaggagcgctggaagtgtgacggagacaacgattgcctggacaacagtgatgaggccccagccctctgccatcagcacacctgcccctcggaccgattcaagtgcgagaacaaccggtgcatccccaaccgctggctctgcgacggggacaatgactgtgggaacagtgaagatgagtccaatgccacttgttcagcccgcacctgcccccccaaccagttctcctgtgccagtggccgctgcatccccatctcctggacgtgtgatctggatgacgactgtggggaccgctctgatgagtctgcttcgtgtgcctatcccacctgcttccccctgactcagtttacctgcaacaatggcagatgtatcaacatcaactggagatgcgacaatgacaatgactgtggggacaacagtgacgaagccggctgcagccactcctgttctagcacccagttcaagtgcaacagcgggcgttgcatccccgagcactggacctgcgatggggacaatgactgcggagactacagtgatgagacacacgccaactgcaccaaccaggccacgaggccccctggtggctgccacactgatgagttccagtgccggctggatggactatgcatccccctgcggtggcgctgcgatggggacactgactgcatggactccagcgatgagaagagctgtgagggagtgacccacgtctgcgatcccagtgtcaagtttggctgcaaggactcagctcggtgcatcagcaaagcgtgggtgtgtgatggcgacaatgactgtgaggataactcggacgaggagaactgcgagtccctggcctgcaggccaccctcgcacccttgtgccaacaacacctcagtctgcctgccccctgacaagctgtgtgatggcaacgacgactgtggcgacggctcagatgagggcgagctctgcgaccagtgctctctgaataacggtggctgcagccacaactgctcagtggcacctggcgaaggcattgtgtgttcctgccctctgggcatggagctggggcccgacaaccacacctgccagatccagagctactgtgccaagcatctcaaatgcagccaaaagtgcgaccagaacaagttcagcgtgaagtgctcctgctacgagggctgggtcctggaacctgacggcgagagctgccgcagcctggaccccttcaagccgttcatcattttctccaaccgccatgaaatccggcgcatcgatcttcacaaaggagactacagcgtcctggtgcccggcctgcgcaacaccatcgccctggacttccacctcagccagagcgccctctactggaccgacgtggtggaggacaagatctaccgcgggaagctgctggacaacggagccctgactagtttcgaggtggtgattcagtatggcctggccacacccgagggcctggctgtagactggattgcaggcaacatctactgggtggagagtaacctggatcagatcgaggtggccaagctggatgggaccctccggaccaccctgctggccggtgacattgagcacccaagggcaatcgcactggatccccgggatgggatcctgttttggacagactgggatgccagcctgccccgcattgaggcagcctccatgagtggggctgggcgccgcaccgtgcaccgggagaccggctctgggggctggcccaacgggctcaccgtggactacctggagaagcgcatcctttggattgacgccaggtcagatgccatttactcagcccgttacgacggctctggccacatggaggtgcttcggggacacgagttcctgtcgcacccgtttgcagtgacgctgtacgggggggaggtctactggactgactggcgaacaaacacactggctaaggccaacaagtggaccggccacaatgtcaccgtggtacagaggaccaacacccagccctttgacctgcaggtgtaccacccctcccgccagcccatggctcccaatccctgtgaggccaatgggggccagggcccctgctcccacctgtgtctcatcaactacaaccggaccgtgtcctgcgcctgcccccacctcatgaagctccacaaggacaacaccacctgctatgagtttaagaagttcctgctgtacgcacgtcagatggagatccgaggtgtggacctggatgctccctactacaactacatcatctccttcacggtgcccgacatcgacaacgtcacagtgctagactacgatgcccgcgagcagcgtgtgtactggtctgacgtgcggacacaggccatcaagcgggccttcatcaacggcacaggcgtggagacagtcgtctctgcagacttgccaaatgcccacgggctggctgtggactgggtctcccgaaacctgttctggacaagctatgacaccaataagaagcagatcaatgtggcccggctggatggctccttcaagaacgcagtggtgcagggcctggagcagccccatggccttgtcgtccaccctctgcgtgggaagctctactggaccgatggtgacaacatcagcatggccaacatggatggcagcaatcgcaccctgctcttcagtggccagaagggccccgtgggcctggctattgacttccctgaaagcaaactctactggatcagctccgggaaccataccatcaaccgctgcaacctggatgggagtgggctggaggtcatcgatgccatgcggagccagctgggcaaggccaccgccctggccatcatgggggacaagctgtggtgggctgatcaggtgtcggaaaagatgggcacatgcagcaaggctgacggctcgggctccgtggtccttcggaacagcaccaccctggtgatgcacatgaaggtctatgacgagagcatccagctggaccataagggcaccaacccctgcagtgtcaacaacggtgactgctcccagctctgcctgcccacgtcagagacgacccgctcctgcatgtgcacagccggctatagcctccggagtggccagcaggcctgcgagggcgtaggttcctttctcctgtactctgtgcatgagggaatcaggggaattcccctggatcccaatgacaagtcagatgccctggtcccagtgtccgggacctcgctggctgtcggcatcgacttccacgctgaaaatgacaccatctactgggtggacatgggcctgagcacgatcagccgggccaagcgggaccagacgtggcgtgaagacgtggtgaccaatggcattggccgtgtggagggcattgcagtggactggatcgcaggcaacatctactggacagaccagggctttgatgtcatcgaggtcgcccggctcaatggctccttccgctacgtggtgatctcccagggtctagacaagccccgggccatcaccgtccacccggagaaagggtacttgttctggactgagtggggtcagtatccgcgtattgagcggtctcggctagatggcacggagcgtgtggtgctggtcaacgtcagcatcagctggcccaacggcatctcagtggactaccaggatgggaagctgtactggtgcgatgcacggacagacaagattgaacggatcgacctggagacaggtgagaaccgcgaggtggttctgtccagcaacaacatggacatgttttcagtgtctgtgtttgaggatttcatctactggagtgacaggactcatgccaacggctctatcaagcgcgggagcaaagacaatgccacagactccgtgcccctgcgaaccggcatcggcgtccagcttaaagacatcaaagtcttcaaccgggaccggcagaaaggcaccaacgtgtgcgcggtggccaatggcgggtgccagcagctgtgcctgtaccggggccgtgggcagcgggcctgcgcctgtgcccacgggatgctggctgaagacggagcatcgtgccgcgagtatgccggctacctgctctactcagagcgcaccattctcaagagtatccacctgtcggatgagcgcaacctcaatgcgcccgtgcagcccttcgaggaccctgagcacatgaagaacgtcatcgccctggcctttgactaccgggcaggcacctctccgggcacccccaatcgcatcttcttcagcgacatccactttgggaacatccaacagatcaacgacgatggctccaggaggatcaccattgtggaaaacgtgggctccgtggaaggcctggcctatcaccgtggctgggacactctctattggacaagctacacgacatccaccatcacgcgccacacagtggaccagacccgcccaggggccttcgagcgtgagaccgtcatcactatgtctggagatgaccacccacgggccttcgttttggacgagtgccagaacctcatgttctggaccaactggaatgagcagcatcccagcatcatgcgggcggcgctctcgggagccaatgtcctgacccttatcgagaaggacatccgtacccccaatggcctggccatcgaccaccgtgccgagaagctctacttctctgacgccaccctggacaagatcgagcggtgcgagtatgacggctcccaccgctatgtgatcctaaagtcagagcctgtccaccccttcgggctggccgtgtatggggagcacattttctggactgactgggtgcggcgggcagtgcagcgggccaacaagcacgtgggcagcaacatgaagctgctgcgcgtggacatcccccagcagcccatgggcatcatcgccgtggccaacgacaccaacagctgtgaactctctccatgccgaatcaacaacggtggctgccaggacctgtgtctgctcactcaccagggccatgtcaactgctcatgccgagggggccgaatcctccaggatgacctcacctgccgagcggtgaattcctcttgccgagcacaagatgagtttgagtgtgccaatggcgagtgcatcaacttcagcctgacctgcgacggcgtcccccactgcaaggacaagtccgatgagaagccatcctactgcaactcccgccgctgcaagaagactttccggcagtgcagcaatgggcgctgtgtgtccaacatgctgtggtgcaacggggccgacgactgtggggatggctctgacgagatcccttgcaacaagacagcctgtggtgtgggcgagttccgctgccgggacgggacctgcatcgggaactccagccgctgcaaccagtttgtggattgtgaggacgcctcagatgagatgaactgcagtgccaccgactgcagcagctacttccgcctgggcgtgaagggcgtgctcttccagccctgcgagcggacctcactctgctacgcacccagctgggtgtgtgatggcgccaatgactgtggggactacagtgatgagcgcgactgcccaggtgtgaaacgccccagatgccctctgaattacttcgcctgccctagtgggcgctgcatccccatgagctggacgtgtgacaaagaggatgactgtgaacatggcgaggacgagacccactgcaacaagttctgctcagaggcccagtttgagtgccagaaccatcgctgcatctccaagcagtggctgtgtgacggcagcgatgactgtggggatggctcagacgaggctgctcactgtgaaggcaagacgtgcggcccctcctccttctcctgccctggcacccacgtgtgcgtccccgagcgctggctctgtgacggtgacaaagactgtgctgatggtgcagacgagagcatcgcagctggttgcttgtacaacagcacttgtgacgaccgtgagttcatgtgccagaaccgccagtgcatccccaagcacttcgtgtgtgaccacgaccgtgactgtgcagatggctctgatgagtcccccgagtgtgagtacccgacctgcggccccagtgagttccgctgtgccaatgggcgctgtctgagctcccgccagtgggagtgtgatggcgagaatgactgccacgaccagagtgacgaggctcccaagaacccacactgcaccagccaagagcacaagtgcaatgcctcgtcacagttcctgtgcagcagtgggcgctgtgtggctgaggcactgctctgcaacggccaggatgactgtggcgacagctcggacgagcgtggctgccacatcaatgagtgtctcagccgcaagctcagtggctgcagccaggactgtgaggacctcaagatcggcttcaagtgccgctgtcgccctggcttccggctgaaggacgacggccggacgtgtgctgatgtggacgagtgcagcaccaccttcccctgcagccagcgctgcatcaacactcatggcagctataagtgtctgtgtgtggagggctatgcaccccgcggcggcgacccccacagctgcaaggctgtgactgacgaggaaccgtttctgatcttcgccaaccggtactacctgcgcaagctcaacctggacgggtccaactacacgttacttaagcagggcctgaacaacgccgttgccttggattttgactaccgagagcagatgatctactggacagatgtgaccacccagggcagcatgatccgaaggatgcaccttaacgggagcaatgtgcaggtcctacaccgtacaggcctcagcaaccccgatgggctggctgtggactgggtgggtggcaacctgtactggtgcgacaaaggccgggacaccatcgaggtgtccaagctcaatggggcctatcggacggtgctggtcagctctggcctccgtgagcccagggctctggtggtggatgtgcagaatgggtacctgtactggacagactggggtgaccattcactgatcggccgcatcggcatggatgggtccagccgcagcgtcatcgtggacaccaagatcacatggcccaatggcctgacgctggactatgtcactgagcgcatctactgggccgacgcccgcgaggactacattgaatttgccagcctggatggctccaatcgccacgttgtgctgagccaggacatcccgcacatctttgcactgaccctgtttgaggactacgtctactggaccgactgggaaacaaagtccattaaccgagcccacaagaccacgggcaccaacaaaacgctcctcatcagcacgctgcaccggcccatggacctgcatgtcttccatgccctgcgccagccagacgtgcccaatcacccctgcaaggtcaacaatggtggctgcagcaacctgtgcctgctgtcccccgggggagggcacaaatgtgcctgccccaccaacttctacctgggcagcgatgggcgcacctgtgtgtccaactgcacggctagccagtttgtatgcaagaacgacaagtgcatccccttctggtggaagtgtgacaccgaggacgactgcggggaccactcagacgagcccccggactgccctgagttcaagtgccggcccggacagttccagtgctccacaggtatctgcacaaaccctgccttcatctgcgatggcgacaatgactgccaggacaacagtgacgaggccaactgtgacatccacgtctgcttgcccagtcagttcaaatgcaccaacaccaaccgctgtattcccggcatcttccgctgcaatgggcaggacaactgcggagatggggaggatgagagggactgccccgaggtgacctgcgcccccaaccagttccagtgctccattaccaaacggtgcatcccccgggtctgggtctgcgaccgggacaatgactgtgtggatggcagtgatgagcccgccaactgcacccagatgacctgtggtgtggacgagttccgctgcaaggattcgggccgctgcatcccagcgcgttggaagtgtgacggagaggatgactgtggggatggctcggatgagcccaaggaagagtgtgatgaacgcacctgtgagccataccagttccgctgcaagaacaaccgctgcgtgcccggccgctggcagtgcgactacgacaacgattgcggtgacaactccgatgaagagagctgcacccctcggccctgctccgagagtgagttctcctgtgccaacggccgctgcatcgcggggcgctggaaatgcgatggagaccacgactgcgcggacggctcggacgagaaagactgcaccccccgctgtgacatggaccagttccagtgcaagagcggccactgcatccccctgcgctggcgctgtgacgcagacgccgactgcatggacggcagcgacgaggaggcctgcggcactggcgtgcggacctgccccctggacgagttccagtgcaacaacaccttgtgcaagccgctggcctggaagtgcgatggcgaggatgactgtggggacaactcagatgagaaccccgaggagtgtgcccggttcgtgtgccctcccaaccggcccttccgttgcaagaatgaccgcgtctgtctgtggatcgggcgccaatgcgatggcacggacaactgtggggatgggactgatgaagaggactgtgagccccccacagcccacaccacccactgcaaagacaagaaggagtttctgtgccggaaccagcgctgcctctcctcctccctgcgctgcaacatgttcgatgactgcggggacggctctgacgaggaggactgcagcatcgaccccaagctgaccagctgcgccaccaatgccagcatctgtggggacgaggcacgctgcgtgcgcaccgagaaagcggcctactgtgcctgccgctcgggcttccacaccgtgcccggccagcccggatgccaagacatcaacgagtgcctgcgcttcggcacctgctcccagctctgcaacaacaccaagggcggccacctctgcagctgcgctcggaacttcatgaagacgcacaacacctgcaaggccgaaggctctgagtaccaggtcctgtacatcgctgatgacaatgagatccgcagcctgttccccggccacccccattcggcttacgagcaggcattccagggtgacgagagtgtccgcattgatgctatggatgtccatgtcaaggctggccgtgtctattggaccaactggcacacgggcaccatctcctaccgcagcctgccacctgctgcgcctcctaccacttccaaccgccaccggcgacagattgaccggggtgtcacccacctcaacatttcagggctgaagatgcccagaggcatcgccatcgactgggtggccggaaacgtgtactggaccgactcgggccgagatgtgattgaggtggcgcagatgaagggcgagaaccgcaagacgctcatctcgggcatgattgacgagccccacgccattgtggtggacccactgagggggaccatgtactggtcagactggggcaaccaccccaagattgagacggcagcgatggatgggacgcttcgggagacactggtgcaggacaacattcagtggcccacaggcctggccgtggattatcacaatgagcggctgtactgggcagacgccaagctttcagtcatcggcagcatccggctcaatggcacggaccccattgtggctgctgacagcaaacgaggcctaagtcaccccttcagcatcgacgtctttgaggattacatctatggtgtcacctacatcaataatcgtgtcttcaagatccataagtttggccacagccccttggtcaacctgacagggggcctgagccacgcctctgacgtggtcctttaccatcagcacaagcagcccgaagtgaccaacccatgtgaccgcaagaaatgcgagtggctctgcctgctgagccccagtgggcctgtctgcacctgtcccaatgggaagcggctggacaacggcacatgcgtgcctgtgccctctccaacgccccccccagatgctccccggcctggaacctgtaacctgcagtgcttcaacggtggcagctgtttcctcaatgcacggaggcagcccaagtgccgctgccaaccccgctacacgggtgacaagtgtgaactggaccagtgctgggagcactgtcgcaatgggggcacctgtgctgcctccccctctggcatgcccacgtgccggtgccccacgggcttcacgggccccaaatgcacccagcaggtgtgtgcgggctactgtgccaacaacagcacctgcactgtcaaccagggcaaccagccccagtgccgatgcctacccggcttcctgggcgaccgctgccagtaccggcagtgctctggctactgtgagaactttggcacatgccagatggctgctgatggctcccgacaatgccgctgcactgcctactttgagggatcgaggtgtgaggtgaacaagtgcagccgctgtctcgaaggggcctgtgtggtcaacaagcagagtggggatgtcacctgcaactgcacggatggccgggtggcccccagctgtctgacctgcgtcggccactgcagcaatggcggctcctgtaccatgaacagcaaaatgatgcctgagtgccagtgcccaccccacatgacagggccccggtgtgaggagcacgtcttcagccagcagcagccaggacatatagcctccatcctaatccctctgctgttgctgctgctgctggttctggtggccggagtggtattctggtataagcggcgagtccaaggggctaagggcttccagcaccaacggatgaccaacggggccatgaacgtggagattggaaaccccacctacaagatgtacgaaggcggagagcctgatgatgtgggaggcctactggacgctgactttgccctggaccctgacaagcccaccaacttcaccaaccccgtgtatgccacactctacatggggggccatggcagtcgccactccctggccagcacggacgagaagcgagaactcctgggccggggccctgaggacgagataggggaccccttggcatagggccctgccccgtcggactgcccccagaaagcctcctgccccctgccagtgaagtccttcagtgagcccctccccagccagcccttccctggccccgccggatgtataaatgtaaaaatgaaggaattacattttatatgtgagcgagcaagccggcaagcgagcacagtattatttctccatcccctccctgcctgctccttggcacccccatgctgccttcagggagacaggcagggagggcttggggctgcacctcctaccctcccaccagaacgcaccccactgggagagctggtggtgcagccttcccctccctgtataagacactttgccaaggctctcccctctcgccccatccctgcttgcccgctcccacagcttcctgagggctaattctgggaagggagagttctttgctgcccctgtctggaagacgtggctctgggtgaggtaggcgggaaaggatggagtgttttagttcttgggggaggccaccccaaaccccagccccaactccaggggcacctatgagatggccatgctcaacccccctcccagacaggccctccctgtctccagggcccccaccgaggttcccagggctggagacttcctctggtaaacattcctccagcctcccctcccctggggacgccaaggaggtgggccacacccaggaagggaaagcgggcagccccgttttggggacgtgaacgttttaataatttttgctgaattcctttacaactaaataacacagatattgttataaataaaattgtaaaaaaaaaaaaaaaaaaaaa

SEQ ID NO: 6 - DNA, 14907 bp, Mus musculus
agtcaggggagcagcggtgcgagctccaggccagtgcactgaggaggcggaaacgggggagcccctagtgctccatcaggcccctaccaaggcacccccatcgggtccacgccccccaccccccaccccgcctcctcccaattgtgcatttttgcagccagaggcggctccgagatggggctgtgagcttcgccctgggagggggagaggagcgaggagtaaagcaggggtgaagggttcgaatttgggggcagggggcgcacccgcgtcagcaggcccttcccagggggctcggaactgtaccatttcacctatgcccctggttcgctttgcttaaggaaaggataagaatagaagagtcggggagaggaagataaagggggaccccccaattggggggggcgaggacaagaagtaacaggaccagagggtgggggctgctgtttgcatcggcccacaccatgctgaccccgccgttgctgctgctgctgccgctgctttcagctctggtctccggggccactatggatgcccctaaaacttgcagccctaagcagtttgcctgcagagaccaaatcacctgtatctcaaagggctggcggtgtgacggtgaaagagattgccccgacggctctgatgaagcccctgagatctgtccacagagtaaagcccagagatgcccgccaaatgagcacagttgtctggggactgagctatgtgtccccatgtctcgtctctgcaacgggatccaggactgcatggatggctcagacgagggtgctcactgccgagagctccgagccaactgttctcgaatgggttgtcaacaccattgtgtacctacacccagtgggcccacgtgctactgtaacagcagcttccagctgcaggcagatggcaagacgtgcaaagattttgacgagtgttccgtgtatggcacctgcagccagctttgcaccaacacagatggctccttcacatgtggctgtgttgaaggctacctgctgcaaccggacaaccgctcctgcaaggccaagaatgagccagtagatcggccgccagtgctactgattgccaactctcagaacatcctagctacgtacctgagtggggcccaagtgtctaccatcacacccaccagcacccgacaaaccacggccatggacttcagttatgccaatgagaccgtatgctgggtgcacgttggggacagtgctgcccagacacagctcaagtgtgcccggatgcctggcctgaagggctttgtggatgagcataccatcaacatctccctcagcctgcaccacgtggagcagatggcaatcgactggctgacgggaaacttctactttgtcgacgacattgacgacaggatctttgtctgtaaccgaaacggggacacctgtgtcactctgctggacctggaactctacaaccccaaaggcatcgccttggaccccgccatggggaaggtgttcttcactgactacgggcagatcccaaaggtggagcgctgtgacatggatggacagaaccgcaccaagctggtggatagcaagatcgtgtttccacacggcatcaccctggacctggtcagccgcctcgtctactgggcggacgcctacctagactacatcgaggtggtagactacgaagggaagggtcggcagaccatcatccaaggcatcctgatcgagcacctgtacggcctgaccgtgtttgagaactatctctacgccaccaactcggacaatgccaacacgcagcagaagacgagcgtgatccgagtgaaccggttcaacagtactgagtaccaggtcgtcacccgtgtggacaagggtggtgccctgcatatctaccaccagcgacgccagccccgagtgcggagtcacgcctgtgagaatgaccagtacgggaagccaggtggctgctccgacatctgcctcctggccaacagtcacaaggcaaggacctgcaggtgcaggtctggcttcagcctgggaagtgatgggaagtcttgtaagaaacctgaacatgagctgttcctcgtgtatggcaagggccgaccaggcatcattagaggcatggacatgggggccaaggtcccagatgagcacatgatccccatcgagaaccttatgaatccacgcgctctggacttccacgccgagaccggcttcatctactttgctgacaccaccagctacctcattggccgccagaaaattgatggcacggagagagagactatcctgaaggatggcatccacaatgtggagggcgtagccgtggactggatgggagacaatctttactggactgatgatggccccaagaagaccattagtgtggccaggctggagaaagccgctcagacccggaagactctaattgagggcaagatgacacaccccagggccattgtagtggatccactcaatgggtggatgtactggacagactgggaggaggaccccaaggacagtcggcgagggcggctcgagagggcttggatggacggctcacaccgagatatctttgtcacctccaagacagtgctttggcccaatgggctaagcctggatatcccagccggacgcctctactgggtggatgccttctatgaccgaattgagaccatactgctcaatggcacagaccggaagattgtatatgagggtcctgaactgaatcatgccttcggcctgtgtcaccatggcaactacctcttttggaccgagtaccggagcggcagcgtctaccgcttggaacggggcgtggcaggcgcaccgcccactgtgacccttctgcgcagcgagagaccgcctatctttgagatccgaatgtacgacgcgcagcagcagcaagtgggtaccaacaaatgccgggtaaataacggaggctgcagcagcctgtgcctcgccacccccgggagccgccagtgtgcctgtgccgaggaccaggtgttggacacagatggtgtcacctgcttggcgaacccatcctacgtgcccccaccccagtgccagccgggcgagtttgcctgtgccaacaaccgctgcatccaggagcgctggaagtgtgacggagacaacgactgtctggacaacagcgatgaggccccagcactgtgccatcaacacacctgtccctcggaccgattcaagtgtgagaacaaccggtgtatccccaaccgctggctctgtgatggggataatgattgtggcaacagcgaggacgaatccaatgccacgtgctcagcccgcacctgtccacccaaccagttctcctgtgccagtggccgatgcattcctatctcatggacctgtgatctggatgatgactgtggggaccggtccgatgagtcagcctcatgcgcctaccccacctgcttccccctgactcaatttacctgcaacaatggcagatgtattaacatcaactggcggtgtgacaacgacaatgactgtggggacaacagcgacgaagccggctgcagtcactcctgctccagtacccagttcaagtgcaacagtggcagatgcatccccgagcactggacgtgtgatggggacaatgattgtggggactacagcgacgagacacacgccaactgtaccaaccaggctacaagacctcctggtggctgccactcggatgagttccagtgccgcctagatggcctgtgcatccccctgaggtggcgctgcgacggggacaccgactgcatggattccagcgatgagaagagctgtgagggcgtgacccatgtttgtgacccgaatgtcaagtttggctgcaaggactccgcccggtgcatcagcaaggcgtgggtgtgtgatggcgacagcgactgtgaagataactccgacgaggagaactgtgaggccctggcctgcaggccaccctcccatccctgcgccaacaacacctctgtctgcctgcctcctgacaagctgtgcgacggcaaggatgactgtggagacggctcggatgagggcgagctctgtgaccagtgttctctgaataatggtggctgtagtcacaactgctcagtggcccctggtgaaggcatcgtgtgctcttgccctctgggcatggagctgggctctgacaaccacacctgccagatccagagctactgtgccaagcacctcaaatgcagccagaagtgtgaccagaacaagttcagtgtgaagtgctcctgctacgagggctgggtcttggagcctgacggggaaagctgccgcagtctggatcccttcaaaccgttcatcatcttctccaaccgccacgagatcaggcgcattgaccttcacaagggggactacagcgtcctagtgcctggcctgcgcaacactattgccctggacttccacctcagccagagtgccctctactggaccgacgtggtagaggacaagatctaccgtgggaaactcctggacaacggagccctgaccagctttgaggtggtgattcagtatggcttggccacaccagagggcctggctgtagattggattgcaggcaacatctactgggtggagagcaacctggaccagatcgaagtggccaagctggacggaaccctccgaaccactctgctggcgggtgacattgagcacccgagggccatcgctctggaccctcgggatgggattctgttttggacagactgggatgccagcctgccacgaatcgaggctgcgtccatgagtggggctggccgccgaaccatccaccgggagacaggctctgggggctggcccaacgggctcaccgtggattacctggagaagcgcatcctctggattgatgctaggtcagatgccatctattcagcccggtatgacggctccggccacatggaggtgcttcggggacacgagttcctgtcacacccatttgccgtgacactgtacggtggggaggtgtactggaccgactggcgaacaaatacactggctaaggccaacaagtggactggccacaacgtcaccgtggtacagaggaccaacacccagcccttcgacctgcaggtgtatcacccttcccggcagcccatggctccaaacccatgtgaggccaatggcggccggggcccctgttcccatctgtgcctcatcaactacaaccggaccgtctcctgcgcctgtccccacctcatgaagctgcacaaggacaacaccacctgctatgagtttaagaagttcctgctgtacgcacgtcagatggagatccggggcgtggacctggatgccccgtactacaattatatcatctccttcacggtgcctgatatcgacaatgtcacggtgctggactatgatgcccgagagcagcgagtttactggtctgatgtgcggactcaagccatcaaaagggcatttatcaacggcactggcgtggagaccgttgtctctgcagacttgcccaacgcccacgggctggctgtggactgggtctcccgaaatctgttttggacaagttacgacaccaacaagaagcagattaacgtggcccggctggacggctccttcaagaatgcggtggtgcagggcctggagcagccccacggcctggtcgtccacccgcttcgtggcaagctctactggactgatggggacaacatcagcatggccaacatggatgggagcaaccacactctgctcttcagtggccagaagggccctgtggggttggccattgacttccctgagagcaaactctactggatcagctctgggaaccacacaatcaaccgttgcaatctggatgggagcgagctggaggtcatcgacaccatgcggagccagctgggcaaggccactgccctggccatcatgggggacaagctgtggtgggcagatcaggtgtcagagaagatgggcacgtgcaacaaagccgatggctctgggtccgtggtgctgcggaacagtaccacgttggttatgcacatgaaggtgtatgacgagagcatccagctagagcatgagggcaccaacccctgcagtgtcaacaacggagactgttcccagctctgcctgccaacatcagagacgactcgctcctgtatgtgtacagccggttacagcctccggagcggacagcaggcctgtgagggtgtgggctcttttctcctgtactctgtacatgagggaattcgggggattccactagatcccaatgacaagtcggatgccctggtcccagtgtccggaacttcactggctgtcggaatcgacttccatgccgaaaatgacactatttattgggtggatatgggcctaagcaccatcagcagggccaagcgtgaccagacatggcgagaggatgtggtgaccaacggtattggccgtgtggagggcatcgcggtggactggatcgcaggcaacatatactggacggaccagggcttcgatgtcatcgaggttgcccggctcaatggctcttttcgttatgtggtcatttcccagggtctggacaagcctcgggccatcactgtccacccagagaaggggtacttgttctggaccgagtggggtcattacccacgtattgagcggtctcgccttgatggcacagagagagtggtgttggttaatgtcagcatcagctggcccaatggcatctcagtagactatcagggcggcaagctctactggtgtgatgctcggatggacaagatcgagcgcatcgacctggaaacgggcgagaaccgggaggtggtcctgtccagcaataacatggatatgttctccgtgtccgtgtttgaggacttcatctactggagtgacagaactcacgccaatggctccatcaagcgcggctgcaaagacaatgctacagactccgtgcctctgaggacaggcattggtgttcagcttaaagacatcaaggtcttcaacagggacaggcagaagggtaccaatgtgtgcgcggtagccaacggcgggtgccagcagctctgcttgtatcggggtggcggacagcgagcctgtgcctgtgcccacgggatgctggcagaagacggggcctcatgccgagagtacgctggctacctgctctactcagagcggaccatcctcaagagcatccacctgtcggatgagcgtaacctcaacgcaccggtgcagccctttgaagaccccgagcacatgaaaaatgtcatcgccctggcctttgactaccgagcaggcacctccccggggacccctaaccgcatcttcttcagtgacatccactttgggaacatccagcagatcaatgacgatggctcgggcaggaccaccatcgtggaaaatgtgggctctgtggaaggcctggcctatcaccgtggctgggacacactgtactggacaagctacaccacatccaccatcacccgccacaccgtggaccagactcgcccaggggccttcgagagggagacagtcatcaccatgtccggagacgaccacccgagagcctttgtgctggatgagtgccagaacctgatgttctggaccaattggaacgagctccatccaagcatcatgcgggcagccctatccggagccaacgtcctgaccctcattgagaaggacatccgcacgcccaatgggttggccatcgaccaccgggcggagaagctgtacttctcggatgccaccttggacaagatcgagcgctgcgagtacgacggctcccaccgctatgtgatcctaaagtcggagcccgtccacccctttgggttggcggtgtacggagagcacattttctggactgactgggtgcggcgggctgtgcagcgagccaacaagtatgtgggcagcgacatgaagctgcttcgggtggacattccccagcaacccatgggcatcatcgccgtggccaacgacaccaacagctgtgaactctccccctgccgtatcaacaatggaggctgccaggatctgtgtctgctcacccaccaaggccacgtcaactgttcctgtcgagggggccggatcctccaggaggacttcacctgccgggctgtgaactcctcttgtcgggcacaagatgagtttgagtgtgccaatggggaatgtatcagcttcagcctcacctgtgatggcgtctcccactgcaaggacaagtccgatgagaagccctcctactgcaactcacgccgctgcaagaagactttccgccagtgtaacaatggtcgctgtgtatccaacatgctgtggtgcaatggggtggatgactgtggggatggctctgatgagattccttgcaacaagactgcctgtggtgtgggtgagttccgctgccgggatgggtcctgcatcgggaactccagtcgctgcaaccagtttgtggattgtgaggatgcctcggatgagatgaattgcagtaccacagactgcagcagctatttccgcctgggcgtgaaaggtgtcctcttccagccgtgcgagcggacatccctgtgctacgcacctagctgggtgtgtgatggcgccaacgactgtggagactacagcgatgaacgtgactgtccaggtgtgaagcgccctaggtgcccgctcaattactttgcctgccccagcgggcgctgtatccccatgagctggacgtgtgacaaggaggatgactgtgagaacggcgaggacgagacccactgcaacaagttctgctcagaggcacagttcgagtgccagaaccaccggtgtatctccaagcagtggctgtgtgacggtagcgatgattgcggggatggctccgatgaggcagctcactgtgaaggcaagacatgtggcccctcctccttctcctgtcccggcacccacgtgtgtgtccctgagcgctggctctgtgatggcgacaaggactgtaccgatggcgcggatgagagtgtcactgctggctgcctgtacaacagcacctgtgatgaccgtgagttcatgtgccagaaccgcttgtgtattcccaagcatttcgtgtgcgaccatgaccgtgactgtgctgatggctctgatgaatcccctgagtgtgagtacccaacctgcggccccaatgaattccgctgtgccaatgggcgttgtctgagctcccgtcagtgggaatgtgatggggagaatgactgtcacgaccacagcgatgaggctcccaagaacccacactgcaccagcccagagcacaaatgcaatgcctcatcacagttcctgtgcagcagcgggcgctgcgtggctgaggcgttgctctgcaacggccaggacgactgtggggacggttcagacgaacgcgggtgccatgtcaacgagtgtctcagccgcaagctcagtggctgcagtcaggactgcgaggacctcaagataggctttaagtgccgctgtcgcccgggcttccggctaaaggacgatggcaggacctgtgccgacctggatgagtgcagcaccaccttcccctgcagccagctctgcatcaacacccacggaagttacaagtgtctgtgtgtggagggctatgcaccccgtggcggtgacccccacagctgcaaagctgtgaccgatgaggagccatttctcatctttgccaaccggtactacctgcggaagctcaacctggacggctccaactacacactgcttaagcagggcctgaacaatgcggtcgccttggactttgactaccgagagcagatgatctactggacggacgtgaccacccagggcagcatgattcgcaggatgcacctcaacggcagcaacgtgcaggttctgcaccggacgggccttagtaacccagatgggctggctgtggactgggtgggtggcaacctgtactggtgtgacaagggcagagataccattgaggtgtccaagcttaacggggcctatcggacagtgctggtcagctctggcctccgggagcccagagctctggtagtggatgtacagaatgggtacctgtactggacagactggggtgaccactcactgatcggccggattggcatggatggatctggccgcagcatcatcgtggacactaagatcacatggcccaatggcctgaccgtggactacgtcacggaacgcatctactgggctgacgcccgtgaggactacatcgagttcgccagcctggatggctccaaccgtcacgttgtgctgagccaagacatcccacacatctttgcgctgaccctatttgaagactacgtctactggacagactgggaaacgaagtccatcaaccgggcccacaagaccacgggtgccaacaaaacactcctcatcagcaccctgcaccggcccatggacttacatgtattccacgccctgcgccagccagatgtgcccaatcacccctgcaaagtcaacaatggtggctgcagcaacctgtgcctgctgtcccctgggggtggtcataaatgcgcctgccccaccaacttctatctgggtggcgatggccgtacctgtgtgtccaactgcacagcaagccagtttgtgtgcaaaaatgacaagtgcatccccttctggtggaagtgtgacacggaggacgactgtggggatcactcagacgagcctccagactgtcccgagttcaagtgccgcccaggccagttccagtgctccaccggcatctgcaccaaccctgccttcatctgtgatggggacaatgactgccaagacaatagtgatgaggccaattgcgacattcacgtctgcttgcccagccaattcaagtgcaccaacaccaaccgctgcattcctggcatcttccgttgcaatgggcaggacaactgcggggacggcgaggatgagcgggattgccctgaggtgacctgcgcccccaaccagttccagtgctccatcaccaagcgctgcatccctcgcgtctgggtctgtgacagggataatgactgtgtggacggcagtgatgagcctgccaactgtacccaaatgacctgtggagtggatgagttccgctgcaaggattctggccgctgcatccccgcgcgctggaagtgtgacggagaagatgactgtggggatggttcagatgagcccaaggaagagtgtgatgagcgcacctgtgagccataccagttccgctgcaaaaacaaccgctgtgtcccaggccgttggcaatgtgactacgacaacgactgcggagataactcggacgaggagagctgcacacctcggccctgctctgagagtgagttttcctgtgccaatggccgctgcatcgctgggcgctggaagtgtgatggggaccatgactgtgccgacggctcagacgagaaagactgcaccccccgctgtgatatggaccagttccagtgcaagagtggccactgcatccccctgcgctggcgctgtgacgcggatgctgactgtatggacggcagtgacgaggaagcctgtggcactggggtgaggacctgcccattggatgagtttcaatgtaacaacaccttgtgcaagccgctggcctggaagtgtgatggagaggacgactgtggggacaactcagatgagaaccccgaggaatgcgcccggttcatctgccctcccaaccggcctttccgctgcaagaatgaccgagtctgcctgtggattgggcgccagtgtgatggcgtggacaactgtggagatgggactgacgaggaggactgtgagccccccacggcccagaacccccactgcaaagacaagaaggagttcctgtgccgaaaccagcgctgtctatcatcctccctgcgctgtaacatgttcgatgactgcggcgatggctccgatgaagaagattgcagcatcgaccccaagctgaccagctgtgccaccaatgccagcatgtgtggggacgaagctcgttgtgtgcgcactgagaaagctgcctactgtgcctgccgctcgggcttccatactgtgccgggccagcccggatgccaggacatcaacgagtgcctgcgctttggtacctgctctcagctctgcaacaacaccaagggaggccacctctgcagctgtgcccgcaacttcatgaagacacacaacacctgcaaagctgaaggctccgagtaccaggtgctatacatcgcggatgacaacgagatccgcagcttgttcccgggccacccccactcagcctacgagcagacattccagggcgatgagagtgtccgcatagatgccatggatgtccatgtcaaggccggccgtgtctactggactaactggcacacgggcacaatctcctacaggagcctgccccctgccgcccctcctaccacttccaaccgccaccggaggcagatcgaccggggtgtcacccacctcaatatttcagggctgaagatgccgaggggtatcgctatcgactgggtggccgggaatgtgtactggaccgattccggccgagacgtgattgaggtggcgcaaatgaagggcgagaaccgcaagacgctcatctcgggcatgattgatgagccccatgccatcgtggtggaccctctgaggggcaccatgtactggtcagactgggggaaccaccccaagattgaaacagcagcgatggatggcacccttcgggagactctcgtgcaagacaacattcagtggcctacagggctggctgtggactatcacaatgaacggctctactgggcagatgccaagctttcggtcatcggcagcatccggctcaacggcactgaccccattgtggctgctgacagcaaacgaggcctaagtcaccccttcagcatcgatgtgtttgaagactacatctacggagtcacttacatcaataatcgtgtcttcaagatccacaagtttggacacagccccttgatcaacctaactgggggcctgagccatgcctctgatgtagtcctttaccatcaacacaagcagcctgaagtgaccaacccctgtgaccgcaagaaatgtgaatggctgtgtctgctgagccccagcgggcctgtctgcacctgtcccaatggaaagaggctggataatggcacctgtgtgcctgtgccctctccaacaccccctccagatgcccctaggcctggaacctgcactctgcagtgcttcaatggtggtagttgtttcctcaatgctcggaggcagcccaagtgccgttgccagccccgttacacaggcgataagtgtgagctggatcagtgctgggaatactgtcacaacggaggcacctgtgcggcttccccatctggcatgcccacgtgccgctgtcccactggcttcacgggccccaaatgcaccgcacaggtgtgtgcaggctactgctctaacaacagcacctgcaccgtcaaccagggcaaccagccccagtgccgatgtctacctggcttcctgggcgaccgttgccagtaccggcagtgctctggcttctgtgagaactttggcacctgtcagatggctgctgatggctcccgacaatgtcgctgcaccgtctactttgagggaccaaggtgtgaggtgaacaagtgtagtcgctgtctccaaggcgcctgtgtggtcaataagcagaccggagatgtcacatgcaactgcactgatggccgggtagcccccagttgtctgacctgcatcgatcactgtagcaatggtggctcctgcaccatgaacagcaagatgatgcctgagtgccagtgcccgccccatatgacaggaccccggtgcgaggagcaggttgttagtcagcaacagcctgggcatatggcctccatcctgatccctctgctgctgcttctcctgctgcttctggtggctggcgtggtgttctggtataagcggcgagtccgaggggctaagggcttccagcaccagcggatgaccaatggggccatgaatgtggaaattggaaaccctacctacaagatgtatgaaggtggagagcccgatgatgtcgggggcctactggatgctgattttgcccttgaccctgacaagcctaccaacttcaccaacccagtgtatgccacgctctacatggggggccacggcagccgccattccctggccagcacggacgagaagcgagaactgctgggccggggacctgaagacgagataggagatcccttggcatagggccctgccccgacggatgtccccagaaagccccctgccacatgagtctttcaatgaaccccctccccagccggcccttctccggccctgccgggtgtacaaatgtaaaaatgaaggaattactttttatatgtgagcgagcaagcgagcaagcacagtattatctctttgcatttccttcctgcctgctcctcagtatcccccccatgctgccttgagggggcggggagggctttgtggctcaaaggtatgaaggagtccacatgttccctaccgagcatacccctggaagctggcggcacggcctccccaccacgcctgtgcaagacactcaacggggctccgtgtcccagctttcctttccttggctctctggggttagttcaggggaggtggagtcctctgctgaccctgtctggaagatttggctctagctgaggaaggagtcttttagttgagggaagtcaccccaaaccccagctcccactttcaggggcacctctcagatggccatgctcagtatcccttccagacaggccctcccctctctagcgccccctctgtggctcctagggctgaacacattctttggtaactgtcccccaagcctcccatccccctgagggccaggaagagtcggggcacaccaaggaagggcaagcgggcagccccattttggggacgtgaacgttttaataatttttgctgaattcctttacaactaaataacacagatattgttataaataaaattgtaaaaaaggaaaaaaaaaagaaaagaaaagaaaagaaaaaaaaaaaaaaaaaa

SEQ ID NO: 7 - DNA, 14900 bp, Macaca mulatta
cagcggtgcgagctccaggcccatgcactgaggaggcggaaacgaggggaacccccagagctccatcaagcccccttgaaaggctcccctacccggtccacgccccccaccccccctccccgcctcctcccaattgtgcatttttgcagccggaggcggctccgagatggggctgtgagcttcgcccggggagggggaaagagcagcgaggagtgaagcgggggggtggggtgaagggtttggatttgggggcaggggcgcaccccagtcagcaggccctccccaaggggctcggaactctacctcttcacccacgcccctggtgcgctttgccgaaggaaagaataagaatagagaaggaggagggggaaaggaggaaaagggggaccccccaattgggggggtgaaggagagaagtagcaggaccagaggggaaggggctgctgcttgcatcagcccacaccatgctgaccccgccgttgctcctgctgctgcccctgctctcagctctggtcgcggccgctatcgacgcccctaagacttgcagccccaagcagtttgcctgcagagatcaaatcacctgtatctcaaagggctggcggtgtgatggtgagagggactgcccagacggatctgacgaggcccctgagatttgtccacagagcaaggcccagcgatgccagccgaacgagcataactgcctgggtaccgagctgtgtgttcccatgtctcgcctctgcaatggagtccaggactgcatggatggctccgatgaggggccccactgccgagagcttcgaggcaactgctctcgcctgggctgccagcaccattgtgtccccacactcgatgggcccacctgctactgcaacagcagctttcagcttcaggcagacagcaagacctgcaaagattttgatgagtgttcagtgtacggcacctgtagccagctatgcaccaacacagatggctcctttatatgtggctgtgtcgaaggatacctgctgcagccggataaccgctcctgcaaggccaagaatgagccagtagaccggccccctgtgctgttgatagccaactcccagaacatcttggccacgtacctgagtggggcccaggtgtctaccatcacacctacgagcactcggcagaccacagccatggacttcagctacgccaatgagaccgtatgctgggtgcatgttggggacaatgctgcccagacgcagctcaagtgtgcccgcatgcctggcctaaagggcttcgtggatgagcacaccatcaacatctccctcagtctgcaccacgtggaacagatggccatcgactggctgacaggcaacttctactttgtggatgacatcgatgataggatctttgtctgcaacagaaatggggacacatgtgtcacattgctagacctggaactctacaaccccaagggcattgccctggatcctgccatggggaaggtgtttttcactgactatgggcagatcccaaaggtggaacgttgtgacatggatgggcagaaccgcaccaagcttgtcgacagcaagattgtgtttcctcacggcatcacgctggacctggtcagccgccttgtctactgggcagatgcctacctggactatattgaagtggtggactatgagggcaaaggccgccagaccatcatccagggcatcctgatcgagcacctgtatggcctgaccgtgtttgagaattacctctatgccaccaactcggacaatgccaatgcccagcagaagacgagtgtgatccgtgtgaaccgctttaatagcaccgagtaccaggttgtcacccgggtggacaagggtggtgccctccacatctaccaccagcggcgtcagccccgagtgaggagccatgcctgtgaaaacgaccagtacgggaagccgggtggctgctctgacatctgcctactggccaatagccacaaggcgaggacctgccgctgccgctccggcttcagcctgggcagtgatgggaagtcatgcaagaagccggagcacgagctgttcctcgtgtatggcaagggccggccaggcatcatccggggcatggatatgggggccaaggtcccggacgaacacatgatccccattgaaaacctcatgaacccccgagccctggacttccacgctgagaccggcttcatctactttgctgacaccaccagctacctcattggccgccagaagatcgatggcactgagcgggagaccatcctgaaggacggcatccacaatgtggagggtgtggctgtggactggatgggggacaatctgtactggacggacgatgggcccaaaaagacaatcagcgtggccaggctggagaaagctgctcagacccgcaagactttaattgagggcaaaatgacacaccccagggctattgtggtagatccgctcaatgggtggatgtactggacagactgggaggaggaccccaaggacagtcggcgtgggcggctggagagggcctggatggatggctcacaccgagacatctttgtcacctccaagacagtgctttggcccaatgggctaagcctggacatcccagctgggcgcctctactgggtggatgccttctacgaccgcattgagacgatactgctcaatggcacagaccggaagattgtgtatgaaggtcctgagctgaaccacgcctttggcctgtgtcaccatggcaactacctcttctggactgagtatcggagtggcagtgtctaccgcttggaacggggtgtaggaggtgcaccccccactgtgacccttctgcgcagtgagcggccccccatctttgagatccgaatgtatgatgcccagcagcagcaagttggcaccaacaaatgccgggtgaacaatggcggctgcagcagcctgtgcttggccacccctgggagccgccagtgcgcctgtgctgaggaccaggtgttggacgcagatggcgtcacttgtttggcgaacccatcctacgtgcctccaccccagtgccagccgggcgagtttgcctgtgccaacagccgctgcatccaggagcgctggaagtgtgatggagacaacgactgcctggacaacagtgatgaggccccagccctctgccatcagcatacctgcccctcggaccgattcaagtgtgagaacaaccggtgcatccccaaccgctggctctgtgacggggacaatgactgtgggaacagtgaagatgagtccaatgccacttgttcagcccgcacctgcccccccaaccagttctcctgtgccagtggccgctgcatccccatctcctggacgtgtgatctggatgatgactgtggggaccgctctgacgagtccgcctcgtgtgcctatcccacctgcttccccctgactcagtttacctgcaacaatggcagatgtatcaacatcaactggcgatgtgacaatgacaatgactgtggggacaacagtgacgaagccggctgcagccactcctgctctagcacccagttcaagtgcaacagcgggcgctgcatccccgagcactggacctgcgatggggacaatgactgcggagattatagtgatgagacgcatgccaactgcaccaaccaggccacgaggccccctggtggctgccacactgatgagttccagtgccggctggatggactgtgcatccccctgcggtggcgctgtgatggggacactgactgcatggactccagcgacgagaagagctgtgagggagtgacccacgtctgcgaccccagtgtcaagtttggctgcaaggactcagctcggtgcatcagcaaagcgtgggtgtgtgatggcgacaacgactgtgaggataactcagatgaggagaactgcgagtccctggcctgcaggccaccctcacacccctgtgccaacaacacctcagtctgcctgccccctgacaagctgtgtgatggcaacgacgactgtggcgacggctcagatgagggcgagctctgcgaccagtgctctctgaataacggtggctgcagccacaactgctcagtggcacctggcgaaggcattgtgtgttcctgccctctgggcatggagctagggcccgacaaccacacctgccagatccagagctactgtgccaagcatctcaaatgcagccaaaagtgcgaccagaacaagttcagcgtgaagtgctcctgctacgagggctgggtcctggagcctgatggggagagctgccgcagcctggaccccttcaagccgttcatcatcttctccaaccggcatgagatccggcgcatcgatcttcacaaaggagactacagcgtcctggtacccggcctgcgcaacaccatcgccctggactttcacctcagccagagcgccctctactggaccgacgtggtggaggacaagatctatcgcgggaagctgctggacaacggagccctgactagttttgaggtggtgattcagtacggcctggccacacccgagggcctggctgtagactggattgcaggcaacatctactgggtggagagtaacctggaccagatcgaggtggccaagctggatgggaccctccggaccactctgctggccggtgacattgagcacccaagggcaatcgcactggatccccgggatgggatcctgttttggacagactgggatgccagcctgccccgcatcgaggcagcctccatgagtggggccgggcgccgcaccgtgcaccgggagaccggctctgggggctggcccaacgggctcactgtggactacctggagaagcgcatcctttggattgacgccaggtcagatgccatttactcagcccgttacgacggctctggccacatggaggtgcttcggggacacgagttcctgtcgcacccatttgcagtgacgctgtacgggggggaggtctactggactgactggcgaacaaacacgctggctaaggccaacaagtggaccggccacaatgtcactgtggtacagaggaccaacacccagccctttgacctgcaggtgtaccacccttcccgccagcccatggctcccaatccctgtgaggccaatgggggccggggcccctgctcccacctgtgtctcatcaactacaaccggaccgtgtcctgcgcctgcccccacctcatgaagctccacaaggacaaaactacttgctatgagtttaagaagttcctgctgtacgcacgtcagatggagatccgaggtgtggacctggatgccccctactacaactacatcatctccttcacggtgcccgacatcgacaacgtcacagtgctagactacgatgcccgtgagcagcgtgtgtactggtctgacgtgcggacacaggccatcaagcgggccttcatcaatggcacaggcgtggagacagtcgtctctgcagacttgccaaatgcccatgggctggctgtggactgggtctcccgaaacctgttctggacaagctatgacaccaataagaagcagatcaatgtggcccggctggatggctccttcaagaacgcagtggtgcagggcctggagcagccccatggccttgtcgtccaccctctgcgtgggaagctctactggaccgatggtgacaacatcagcatggccaacatggacggcagcaatcgcaccctgctcttcagtggccagaagggccccgtgggtctggctattgacttccctgaaagcaaactctactggatcagctccgggaaccataccatcaaccgctgcaacctggatgggagtgggctggaggtcatcgacgccatgcggagccagctgggcaaggccactgccctggccatcatgggggacaagctgtggtgggcagatcaggtgtcggagaagatgggcacatgcagcaaggccgacggctcgggctccatcgtcctgcggaacagcaccaccctggtgatgcacatgaaggtctatgacgagagcatccagctggaccataagggcaccaacccctgcagtgtcaacaacggtgactgctcccagctctgcctgcccacgtcagagacgacccgctcctgcatgtgcacagccggctatagcctccggagtggccagcaggcctgtgagggcgtgggttcctttctcctgtactctgtgcacgaaggaatcaggggaattcctctggatcccaatgacaagtcagatgccctggtcccagtgtccgggacctcgctggctgtcggcatcgacttccatgctgaaaatgacaccatctactgggtggacatgggcctgagcacgatcagccgggccaagcgggaccagacgtggcgtgaagacgtggtgaccaatggcattggccgcgtggagggcatcgcagtggactggatcgcaggcaacatctactggacggaccagggcttcgatgtcatcgaggtcgcccggctcaatggctccttccgctacgtggtgatctcccagggtctagacaagccccgggccatcaccgtccacccagagaaagggtacctgttctggactgagtggggtcagtatccacgtattgagcggtctcggctagatggcacagaacgtgtggtgctggtcaacgtcagcatcagctggcccaatggcatctcagtggactaccaggatgggaagctgtactggtgtgatgcacggacagacaagattgaacggatcgacctggagacgggtgagaaccgcgaggtggttctgtccagcaacaacatggacatgttttcagtgtctgtgtttgaggatttcatctactggagtgacaggactcacgccaacggctctatcaagcgagggagcaaagacaatgccacagactccgtgcccctgcgaaccggcatcggcgtccagcttaaagatatcaaagtcttcaaccgggaccggcagaaaggcacgaacgtgtgcgcggtggccaatggtgggtgccagcagctgtgcctgtaccggggccgtgggcagcgggcctgcgcctgtgcccacgggatgctggctgaagacggagcatcgtgccgcgagtacgccggctacctgctctactcggagcgcaccattctcaagagcatccacctgtcggatgagcgcaacctcaatgcgcccgtgcagcccttcgaggaccctgagcacatgaagaacgtcattgccctggcctttgactaccgggcaggcacctctccgggcacccccaatcgcatcttcttcagcgacatccactttgggaacattcagcagatcaacgacgatggctccaggaggatcaccattgtggagaatgtgggctccgtagaaggcctggcctatcaccgtggctgggacactctctattggacaagctacacgacatccaccatcacgcgccacacagtggaccagacccgcccaggggccttcgagcgtgaaaccgtcatcactatgtccggagatgaccacccacgggccttcgtgttggatgagtgccagaacctcatgttctggaccaactggaatgagcagcatcccagcatcatgcgggcagcgctctcgggagccaatgtcctgaccctcatcgagaaggatatccgcacccccaacggcctggccatcgaccaccgtgccgagaagctctacttctctgacgccaccctggacaagattgagcggtgcgagtatgacggctcccaccgctatgtgatcctaaagtcagagcctgtccaccccttcgggctggccgtgtatggggagcacattttctggaccgactgggtgcggcgggcagtgcagcgggccaacaagcacgtgggcagcaacatgaagctgctgcgcgtggacatcccccagcagcccatgggcatcatcgccgtggccaacgacaccaacagctgtgaactctctccatgccgaatcaacaatggtggctgccaggacctgtgtctgctcactcaccagggccatgtcaactgctcgtgccgagggggccgaatcctccaggatgacctcacctgccgagcggtgaattcctcttgccgagcacaagatgagtttgagtgtgccaatggcgagtgcatcaacttcagcctgacctgcgacggcgtcccccactgcaaggacaagtccgatgagaagccatcctactgcaactcccgccgctgcaagaagactttccgccagtgcagcaatgggcgctgtgtgtccaacatgctgtggtgcaacggggccgacgactgtggggatggttctgatgagatcccctgcaacaagacagcctgtggtgtgggcgagttccgctgccgggacgggacctgcatcgggaactccagccgctgcaaccagtttgtggattgtgaggatgcctcagatgagatgaactgcagtgccaccgactgcagcagctacttccgcctgggcgtgaagggcgtgctcttccagccctgtgagcggacctcgctctgctacgcacccagctgggtgtgtgacggcgccaacgactgcggggactacagtgatgagcgcgactgcccaggtgtgaaacgccccagatgccccctgaattacttcgcctgccctagtgggcgctgcatccccatgagctggacgtgtgacaaggaggatgactgtgaacacggcgaggacgagacccactgcaacaagttctgctcagaggcccagtttgagtgccagaaccatcgctgcatctccaagcagtggctgtgtgacggcagcgatgactgtggggacggctcggacgaggctgctcactgtgaaggcaagacgtgcggcccctcctccttctcctgccctggcacccacgtgtgcgtccccgagcgctggctctgtgacggtgacaaagactgtgctgatggtgcagacgagagcatcgcagctggttgcttgtacaacagcacctgcgacgaccgtgagttcatgtgccagaaccgccagtgcatccccaagcacttcgtgtgcgaccatgaccgtgactgtgcagatggctccgatgagtcccccgagtgtgagtacccgacctgcggccccagtgagttccgctgtgccaatgggcgctgtctgagctcccgccagtgggagtgtgatggcgagaatgactgccacgaccagagtgacgaggctcccaagaacccacactgcaccagcccagagcacaagtgcaatgcctcgtctcagttcctgtgcagcagcgggcgctgtgtggctgaggtactgctctgcaatggccaggatgactgtggtgacggctcggatgagcgtggctgccacatcaacgagtgtctcagccacaagctcagtggctgcagccaggactgtgaggacctcaagattggcttcaagtgccgctgtcgccctggcttccggctgaaggacgacggccggacatgtgccgatgtggatgagtgcagcaccaccttcccctgcagccagcgctgcatcaacacccatggcagctataagtgtctgtgtgtggagggctacgcaccccgcggcggcgacccccacagctgcaaggctgtgactgacgaggaaccgtttctgatctttgccaaccggtactacctacgcaagctcaacctggatgggtccaactacacgttacttaagcagggcctgaacaatgccgttgccttggactttgactaccgagagcaaatgatctactggacagatgtgacaacccagggcagcatgatccgaaggatgcaccttaatgggagcaacgtgcaggtcctacaccgtacaggcctcagcaaccccgacgggctggctgtggactgggtgggtggcaacctgtactggtgcgacaaaggccgggacaccattgaggtgtccaagctcaatggggcctatcggacggtgctggtcagctctggcctccgcgagcccagggctctggtggtggatgtgcagaatgggtacctgtactggacagactggggtgaccactcactgattggccgcatcggcatggatgggtccagtcgcagcgtcattgtggacaccaagatcacatggcccaacggcctgacgctggactatgtcactgagcgcatctactgggctgacgcccgcgaggactacattgagtttgccagcctggatggctccaatcgccacgttgtgctgagccaggacatcccgcacatctttgcactgaccctgtttgaggactacgtctactggaccgactgggaaacaaagtccatcaaccgagcccacaagaccacgggcaccaacaaaacgctcctcatcagcacgctgcaccggcccatggacctgcacgtcttccacgccctgcgccagccggacgtgcccaatcacccctgcaaggtcaacaatggtggctgcagcaacctgtgcctgctgtcccccgggggagggcacaaatgtgcctgccccaccaacttctacctgggcagcgatgggcgcacctgtgtgtccaactgcacagcgagccagtttgtgtgcaagaacgacaagtgcatccccttctggtggaagtgtgacaccgaggacgactgcggggaccactcagatgagcccccggactgccccgagttcaagtgccggcccggacagttccagtgctccacaggcatctgcacaaaccctgccttcatctgcgatggagacaatgactgccaggacaacagtgacgaggccaactgtgacatccacgtctgcttgcccagtcagttcaaatgtaccaataccaaccgctgtattcccggcatcttccgctgcaacgggcaggacaactgcggagacggggaggacgagagggactgccccgaggtgacctgcgctcccaaccagttccagtgctccattaccaaacggtgcatcccccgggtctgggtctgcgaccgggacaatgactgtgtggatggcagtgatgagcccgccaactgcacccagatgacctgtggcgtggacgagttccgctgcaaggattcgggccgatgcatcccagcgcgctggaagtgtgatggagaggatgactgcggggatggctcagatgagcccaaggaagagtgtgatgagcgcacctgtgagccataccagttccgctgcaagaacaaccgctgcgtgcccggccgctggcagtgtgactacgacaacgattgtggcgacaactccgacgaggagagctgcacccctcgaccctgctccgagagtgagttctcctgtgccaacggccgctgcatcgcggggcgctggaaatgcgatggagaccacgactgcgctgacggctcagacgagaaagactgcaccccccgctgtgacatggaccagttccagtgcaagagcggccactgcatccccctgcgctggcgctgtgacgcagacgctgactgcatggacggcagcgacgaggaggcctgcggcactggcgtgcggacctgccccctggatgagttccagtgcaacaacaccttgtgcaagccgctggcctggaagtgcgatggcgaggatgactgtggggacaactcagatgagaaccccgaggagtgtgcccggttcgtgtgccctcccaaccggcccttccgttgcaagaatgaccgtgtctgtctgtggatcggacgccaatgcgacggcatggacaactgtggggatgggactgatgaagaggactgtgagccccccacggcccagaccacccactgcaaagataagaaggagtttctgtgccggaaccagcgctgcctctcctcctccctacgctgcaacatgttcgacgactgcggggatggctctgacgaggaggactgcagcatcgaccccaagctgaccagctgcgccaccaatgccagcatctgtggggacgaggcacgctgcgtacgcaccgagaaagcagcctactgtgcctgccgctctggcttccacaccgtgcccggccagcccggatgtcaagacatcaacgagtgcctgcgcttcggcacctgctcccagctctgcaacaacaccaagggcggccacctctgcagctgcgctcggaacttcatgaagacgcacaacacctgcaaggctgaaggctctgagtaccaggtcctgtacattgctgatgacaatgagatccgcagcctgttccctgggcacccccattcggcttacgagcaggcattccagggcgacgagagcgtccgcattgatgccatggatgtccatgtcaaggctggccgtgtctattggaccaactggcacacgggcaccatctcctaccgcagcctgccacctgctgcgcctcctaccacttccaaccgccaccggcgacagattgaccggggtgtcacccacctcaacatttcagggctgaagatgcccagaggcattgccatcgattgggtggccggaaacgtgtactggactgactcgggccgagatgtgattgaggtggcacagatgaagggcgagaaccgcaagacactcatctcgggcatgattgatgagccccacgccattgtggtggacccactgaggggcaccatgtactggtcagactggggcaaccaccccaagattgagacagcagcgatggatgggacccttcgggagacactggtgcaggacaacattcagtggcccacaggcctggccgtggattatcacaatgagcggttgtactgggcagatgccaagctttcagtcatcggcagcatccggctcaatggcacggaccccattgtggctgctgacagcaaacgaggcctaagtcaccccttcagcatcgacgtctttgaggattacatctatggtgtcacctacatcaataatcgtgtcttcaagatccataagtttggccacagccccttggtcaacctgacagggggcctgagccatgcctctgatgtggtcctgtaccatcagcacaagcagcccgaagtgaccaacccatgtgaccgcaagaaatgcgagtggctctgcctgctgagccccagtgggcctgtctgcacctgtcccaatgggaaacggctggacaacggcacatgcgtgcctgtgccctctccaacaccccccccagatgctccccggcctggaacctgtaacctgcagtgcttcaacggtggcagctgtttcctcaatgcacggaggcagcccaagtgccgctgccagccccgctacacgggtgacaaatgtgaactggaccaatgctgggagcactgtcgcaatgggggcacctgtgctgcctctccctctggcatgcccacgtgccggtgccccacgggcttcacgggccccaaatgcacccagcaggtgtgtgcaggctactgtgccaacaacagcacctgcactgtcaaccagggcaaccagccccagtgccgatgcctacccggcttcctgggcgaccgctgccagtaccggcagtgctctggctactgtgagaactttggcacatgccagatggccgctgatggctcccgacaatgtcgctgcactgcctactttgagggactgaggtgtgaggtgaacaagtgcagccgctgtctcgaaggggcctgtgtggtcaacaagcagagtggggatgtcacctgcaactgcacggacggccgggtggcccccagctgtctgacctgcatcggccactgcagcaatggcggctcctgcaccatgaacagcaaaatgatgcctgagtgccagtgcccaccccacatgacagggccccggtgtgaggagcacgtcttcagccagcagcagccaggacatatagcctccatcctaatccctctgctcttgctgctgctggtgcttctggtggccggagtggtattctggtataagcggcgagtccaaggggctaagggcttccagcaccagcggatgaccaacggggccatgaatgtggagattgggaaccccacctacaagatgtacgaaggcggagagcctgatgacgtgggaggcctactggacgccgactttgccctggaccctgacaagcccaccaacttcaccaaccccgtgtatgccacactctacatggggggccatggcagtcgccactccctggccagcacggacgagaagcgagaactcctgggccggggccctgaggacgagataggggaccccttggcatagggccctgccccgtcgcacttcccccagaaagcctcctgccccctgccagtgaagtccttcagtgagcccctccccagccagcccttccccggcctcgccggatgtataaatgtaaaaatgaaggaattacgttttatatgtgagcgagcaagccagcaagcgagcacagtattatttctccatcccctccctgcctgctcctcggcacccccatgctgccttcagggaggcaggcagggagggcttggggctgcacttcctaccctcccaccagaacacaccccaccgggagagctggtggtgcagcctccccctccctgtataagacactttgccaaggctctcccttctcgaccctacccctgcttgcccactcccacagctcccggagggctaattctggggaaggagagttctttgctgcccctgtctggaagacgtggctctgggtgaggtaggcaggaaaggatggagtgttttagttcttgggggaggccaccccaaagcccagccctgactccaggggcacctatgagatggccatgctgaatccccctcccagacaggcccttcccatctccagggcccccactgaggttcccagggctggagacttcctctggtaaacattcccccagcctcccctcccctggggacactgaggaggtgggccacacccaggaagggcaagtgggcagccccgttttggggacgtgaacgttttaataatttttgctgaattcctttacaacgaaataacacagatattgttataaataaaattgtaaaaaaaaaaaaagt

SEQ ID NO: 8 - DNA, 14714 bp, Rattus norvegicus
caccccccaccccgcctcctcccaattgtgcatttttgcagccggaggcggctccgagatggggctgtgagcttcgccctgggagggggagaggagcgaggagtaaagcaggggtgaagggttcgaatttgggggcagggggcgcacccgcgtcagcaggcccttcccagggggctcggaactgtatcatttcacctatgcccctgattcgctttgcttaaggaaaggataagaatagaagagtcagggagaggaagataaagggggaccccccaattggggggggcgaggacaagaagtaacaggaccagagggtgggggctgctgtttccatcggcccacaccatgctgaccccgccgttgctgctgctgctgcccctgctttcagctctggtcgccggggccactatggatgcccctaaaacttgcagccctaagcagtttgcctgcagagaccaaatcacctgtatctcgaagggctggcggtgtgacggggaaagagattgtccggacggctctgatgaagcccccgagatctgtccacagagtaaagcccagagatgcccaccaaatgagcacagttgcctggggaccgagctgtgtgtccccatgtctcgtctctgcaacgggatccaggattgcatggatggctcagatgagggtgctcactgccgagagctccgtgtcaactgttctcgaatgggctgtcagcaccattgcgtccctacgcccagtgggcccacatgctactgtaataacagcttccagcttcaggcagacggcaagacatgcaaagattttgacgaatgctctgtgtatggcacttgcagccagctttgcaccaacacagatggctccttcacatgtggctgtgttgaaggttacctgctgcaaccggacaaccgctcatgcaaggccaagaatgagccagtagatcggcccccggtgctactgattgccaactcccagaacatcctagctacgtacctgagcggagcccaggtgtctaccatcacacccaccagcacccgacagaccacagccatggacttcagttatgccaacgagactgtatgctgggtacatgttggggacagtgctgcccagacgcagctcaagtgtgcccggatgcctagcctgaagggcttcgtggatgagcataccatcaacatctccctgagtctgcaccacgttgagcagatggctatcgactggctgactgggaacttctactttgtggatgacatcgatgacaggatctttgtctgtaaccgaaatggggacacctgtgtcactttgctggacctggagctctacaatcccaaaggcatcgccctggaccctgccatggggaaggtgttcttcactgactacgggcagatcccaaaggtggaacgctgtgacatggacggacagaaccgcaccaagctggtcgatagcaagattgtatttccacatggcatcaccctggacctggtcagccgcctcgtgtactgggcggacgcctaccttgactatatcgaggtggtagactatgaaggaaagggccggcagaccatcatccaaggcatcctgattgagcacctctatggcctgactgtgtttgagaactacctctacgccaccaactcagacaacgccaacacccagcagaagacgagcgtgatccgagtgaaccggttcaacagtaccgagtaccaggtggtcacccgtgtggacaagggcggtgccctgcatatctatcaccagcgacgccagccccgagtgcggagtcatgcctgtgagaatgaccagtatgggaagccaggaggctgctctgacatctgcctgctggccaacagccacaaggcaaggacctgcaggtgccggtctggcttcagtctgggaagtgacgggaaatcctgcaagaaacctgaacatgagctgttcctcgtgtatggcaagggccggccaggcatcatccgaggcatggacatgggagccaaggtcccagatgagcacatgatccccatcgagaaccttatgaatccacgggctctggacttccacgctgagactggcttcatctactttgctgacaccaccagctacctcattggccgccagaaaattgatggcacggagagagagaccatcctgaaggacggcatccacaacgtggagggcgtagctgtagactggatgggggacaacctttactggactgatgacggccccaagaagaccattagtgtggccaggctggagaaagctgcccagacacgaaagactctaatcgagggcaagatgacacaccccagggccattgtagtggatccactcaatgggtggatgtactggacagactgggaggaagaccccaaggatagccggcgagggcggcttgagagggcttggatggacggctcacaccgagatatctttgtcacctccaagacagtgctttggcccaatgggctaagcctggatatcccagctgggcgcctctactgggtggatgccttctatgaccgaattgagaccatactgctcaatggcacagaccggaagattgtatacgagggtcctgaactgaatcacgccttcggcctgtgtcaccacggcaactacctcttttggactgagtatcggagcggcagtgtctaccgcttggagcggggtgtggcaggcgcacagcccactgtgacccttctgcgcagcgagcgacctcctatctttgagatccgaatgtacgacgcgcagcagcagcaagtgggtaccaacaaatgccgggtaaataacggaggctgcagcagtctgtgcctagccaccccggggagtcgccagtgcgcctgcgctgaggaccaggtgttggatgcggatggcgtcacctgcctggcgaacccatcctacgtgcccccaccccagtgccagccgggcgagtttgcctgtgccaacaaccgctgcatccaggagcgctggaagtgtgatggagataacgactgtctggacaacagtgatgaggccccggcactgtgccatcaacacacctgtccctcggaccgattcaaatgtgagaacaaccgatgtatccccaaccgctggctctgtgatggggataacgactgtggcaacagcgaggacgagtccaatgccacgtgctcagcgcgcacctgcccacccaaccagttctcctgtgccagtggccgatgcatccctatctcttggacctgtgatcttgatgatgactgtggggaccgctccgatgagtcagcctcatgcgcctaccccacctgtttccccctgactcagtttacctgcaacaatggcagatgcattaacatcaactggcggtgtgacaacgacaatgactgtggagacaatagtgacgaagccggctgcagtcactcctgctccagtacccagttcaagtgcaacagtggcagatgcatccccgagcactggacttgtgacggggacaacgactgtggagactacagtgatgagacccatgcaaactgtaccaaccaggccacaagacctcctggtggctgccactcagatgagttccagtgccggctagatggcctgtgcatccccctgcggtggcgctgtgatggggacactgactgcatggactctagtgatgagaagggctgtgagggggtgacccacgtctgtgatccgaatgtcaagtttggctgcaaggactcagctcggtgcatcagcaaagcatgggtgtgtgatggtgacagtgactgtgaagataactcagacgaggagaactgtgaggccctggcctgcaggccaccgtcacatccctgtgccaacaacacctccgtctgcctgtcccctgataagctgtgtgatggcaaggatgactgtggagatggctccgacgagggcgagctctgtgaccagtgttctctgaataatggtggctgtagtcacaactgctcggtggcccctggtgaaggcattgtgtgctcttgccctctgggcatggagctgggacctgacaaccacacctgccagatccagagctactgtgccaagcacctcaaatgcagccagaagtgcgaccagaacaagttcagtgtgaagtgctcctgctatgagggctgggtcttggaaccagacggggagagctgccgcagcctggatcccttcaaaccgttcatcatcttctccaaccgccatgagatcagacgcattgaccttcacaagggggactacagcgtcctagtgcccggcctgcgcaacaccattgccctggactttcacctcagccagagtgccctctactggaccgatgtggtagaggacaagatctaccgtgggaagctgctggacaacggagcactgaccagctttgaggtggtgattcagtatggcttggccaccccagagggcctggctgtagactggatagcaggcaacatctactgggtggaaagcaacctggaccagatcgaggtggccaagctggatggaaccctccgaaccactctgctggcgggcgacattgagcacccaagggcaattgctctggaccctcgggatgggattctgttttggacagattgggatgccagtctgccccgaattgaagcagcatccatgagtggggccgggcgccgaaccatccaccgagagacaggctctgggggttggcccaacgggctcaccgtggactacctggagaagcgcatcctctggatcgatgccaggtcagatgctatctactcagcccgttatgacggctccggccacatggaggtgctccgggggcatgagttcctgtctcacccgtttgccgtgacactgtatggtggggaggtgtactggactgactggcgaacaaacacactggctaaggccaacaagtggaccggccacaatgtcactgtggtacagaggaccaacacccagcccttcgacctgcaggtgtatcacccttctcggcagcccatggctccaaacccatgtgaggccaatgggggccggggtccctgttcccacctgtgcctcatcaactacaaccggacggtctcctgtgcttgtccccatctcatgaaactccacaatgacaacaccacctgctacgagtttaagaagttcctgctgtacgcacgtcagatggagatccggggtgtggacctggacgccccgtactacaattacatcatctccttcacggtgcccgacattgacaatgtcacagtgctggactatgatgcccgagagcagcgagtttactggtctgacgtgcgaacccaagccatcaaacgggcattcatcaacggcacaggcgtggagaccgttgtctctgcagacttgccaaatgcccatgggctggctgtggactgggtgtcccgaaatctgttctggaccagttatgacaccaacaagaagcagattaacgtggcccggctagatggctccttcaagaatgcggtggtgcagggcctggagcagccccacggcctggttgtccacccgcttcgtggcaagctctactggacggacggggacaatatcagcatggtcaacatggatgggagcaaccggactctgctcttcagtggccagaagggccctgtgggcttagccattgacttccctgagagcaaactctactggatcagctctgggaaccacacgatcaaccgttgcaatctggatgggagtgagctggaggtcatcgacaccatgcgtagccagctgggcaaggccactgccctggccatcatgggggacaagctgtggtgggcagatcaggtgtcagagaagatgggcacatgcaacaaggccgacggctccgggtcggtggtgctgcggaacagcaccacgttggttatgcacatgaaggtgtatgatgagagcatccagctagagcatgagggcaccaacccctgcagtgtcaacaatggagactgctcccagctctgcctgccaacatcagagacaactcgctcctgtatgtgtacagctggttacagcctccggagcggacagcaggcctgtgagggtgtgggttcttttctcctgtattctgtccatgagggaattcgggggatcccactggatcccaatgacaagtcggatgccctggtcccagtgtcgggaacgtcactggctgttggaatcgacttccatgctgaaaatgacactatttattgggtggacatgggtctaagcaccatcagcagggccaagcgtgaccagacatggcgagaggatgtggtgaccaatggcattggccgtgtggagggcatcgcggtggactggatcgcaggcaacatctactggacagaccagggctttgatgtcatcgaggttgcccgactcaatggatctttccgttatgtggtcatttcccagggtctagacaagcctcgggccatcactgtccacccagagaaggggtacttgttctggactgagtggggtcactacccacggattgagcggtctcgccttgacggcacagagagagtggtgctggttaatgtcagcatcagctggcccaatggcatctcagtagactatcagggcggcaagctctactggtgtgatgcccggatggacaagatcgaacgtatcgatctggagacgggtgagaaccgtgaggtggtcctgtccagtaacaacatggacatgttctctgtgtctgtgtttgaggatttcatctactggagtgacagaactcacgccaacggctccatcaagcgtggatgcaaagacaatgccacagactccgtgcctctgagaacgggcattggcgtgcagcttaaagacatcaaggtcttcaacagggacaggcagaagggtaccaacgtgtgcgcagtagccaacggtgggtgccagcaactatgcttatatcggggtggtggacagcgagcctgtgcctgtgcccatggaatgctggcagaagatggggcttcgtgccgagagtatgctggctacctgctctattcagagcgtaccatcctcaagagcatccacctgtcagatgagcgtaacctcaacgcaccggtgcagcctttcgaagaccctgagcacatgaaaaatgtcatcgccctagcttttgactaccgggcaggcacctccccagggacccctaaccgcatcttcttcagtgacatccactttgggaatatccagcagatcaatgacgatggctcggggaggaccaccatcgtggaaaatgtgggctctgtggaaggcctggcctatcacagaggctgggacacactgtactggacaagctacacgacatccaccatcacccgccataccgtggaccagactcgcccaggggcctttgagagggagacggtcatcaccatgtctggagatgatcacccaagggcatttgtgctggacgagtgccagaacctgatgttctggaccaattggaatgagcttcacccaagcatcatgcgggcagccctatctggagccaacgtcctgaccctcatcgagaaggacatccgcacacccaatgggttggccatcgaccaccgggccgagaagctttacttctcggacgccacattggacaagatcgagcgctgtgaatatgatggctcccatcgctatgtgatcctgaagtcagagcccgtccacccctttgggttggcagtgtacggagagcacattttctggactgactgggtgcggcgggctgtgcagcgggccaacaagtatgtgggcagtgacatgaagctgctgcgagtagacatcccccagcagcccatgggcatcatcgctgtggccaatgacaccaacagctgtgaactttccccctgccgtatcaacaatggcggctgtcaggatctgtgtctgctcacccaccaaggccatgtcaactgttcctgtcgagggggccggatcctccaggaggatttcacctgccgggctatgaactcctcttgtcgggcacaagatgagttcgagtgcgccaatggagagtgtatcagcttcagcctcacctgtgatggtgtctcccactgcaaggacaagtctgatgagaagccctcctactgcaactcacgccgctgcaagaagactttccgccagtgcaacaacggccgctgtgtatctaacatgctgtggtgcaatggggtggacgactgtggcgatggctccgatgagattccttgcaacaagaccgcctgcggcgtgggtgaattccgctgccgggatgggtcctgcatcgggaactccagtcgctgcaaccagtttgtggattgtgaggatgcctcggatgagatgaattgcagcgccaccgactgcagcagttatttccgcctgggcgtgaaaggtgtcctcttccagccttgcgagcggacatccctctgctatgcacccagctgggtgtgcgatggtgccaacgactgtggagactacagtgacgagcgtgactgcccaggtgtgaagcgcccacggtgcccactcaattactttgcctgccccagcgggcgctgcatccccatgagctggacgtgtgacaaagaggacgattgtgagaacggcgaggatgagacccactgcaacaagttctgctcggaggcccagtttgagtgccagaaccaccggtgtatctccaagcagtggctgtgtgacggcagcgatgactgcggggacggctccgatgaggcagctcactgtgaaggcaagacttgcggcccctcctccttctcctgtcctggcacccacgtgtgtgtccccgagcgctggctctgtgacggtgacaaggactgtgctgatggcgcggatgagagcatctcagctggctgcctgtacaacagcacctgtgacgaccgtgagttcatgtgccagaaccgcctgtgtattcccaagcattttgtgtgtgaccatgaccgcgactgtgccgatggctctgatgaatcccctgagtgtgaatacccaacctgcggccccaacgaattccgctgcgccaatgggcgttgtctgagctcccgccagtgggagtgtgatggggagaatgactgtcatgaccacagtgatgaggctcccaagaacccacactgcacaagcccagagcacaaatgcaatgcctcatcacagttcctgtgcagcagcgggcgctgcgtggctgaggcgttgctctgcaatggccaggacgactgcggggatggttcagacgaacgcgggtgccacgtcaacgagtgtctcagccgcaagctcagtggctgcagtcaggactgcgaggacctcaagataggctttaagtgccgctgtcgccctggcttccggctaaaggatgatggcagaacctgtgctgatgtggacgagtgcagcaccaccttcccctgcagccagctctgcatcaacacccatggcagttacaagtgtctgtgtgtggagggctatgcaccccgcggtggtgacccccacagctgcaaagctgtgaccgatgaggagccgtttctcatctttgcgaaccggtactacctgcgcaagctcaacttggacggctccaactacacactgcttaagcagggcctgaacaatgcagttgccttggactttgactaccgggggcagatgatctactggacagacgtgacgacccagggcagcatgatccgaaggatgcacctcaatggtagcaacgtgcaggttctgcaccggacaggccttagtaaccccgatgggctggctgtggactgggtgggtggcaacctgtactggtgtgacaagggcagagacactattgaggtgtccaagctcaacggggcctatcggacagtgctggtcagctctggcctccgtgagcccagagctcttgtggtggatgtacagaacgggtacctctactggacagactggggtgaccactcactgatcggtcggattggcatggatgggtctggccgcagtatcattgtggacactaagatcacatggcccaatggcctgactgtggactacgtcacggagcgcatctactgggctgatgcccgtgaggactacatcgagtttgccagcctggatggatccaaccgccatgttgtgctgagccaagacatcccacacatctttgcactgaccctatttgaggattacgtctactggaccgactgggaaacaaagtccatcaaccgggcccataagaccacgggtgccaacaaaaccctcctcatcagcaccctgcaccggcccatggacctacatgtcttccacgccctgcgccagccagatgtgcccaatcacccctgcaaagtcaacaacggtggctgcagcaacctgtgcctgctgtctcctgggggtggtcacaaatgcgcctgccccaccaacttctatctgggtggtgacggccgtacctgtgtgtctaactgcacagcaagccagtttgtatgcaagaatgacaagtgcatccccttctggtggaagtgtgacactgaggacgattgtggggaccactcagacgagcctccagactgtcccgagttcaagtgccgcccaggccagttccagtgctccaccggcatctgcaccaaccctgccttcatctgtgatggggacaatgactgccaagacaatagtgacgaggccaactgtgacatccacgtctgcttgcccagtcaattcaagtgcaccaacaccaaccgctgtatccctggcatcttccgttgcaacgggcaggacaactgtggggacggcgaggatgaacgggattgccctgaggtgacctgtgcccccaaccagttccagtgctctatcaccaagcgctgcatcccccgagtctgggtctgcgacagggacaatgactgtgtggacggaagtgatgaacctgccaactgcacccagatgacctgcggggtggatgagttccgctgcaaggactcgggccgctgcatccctgcacgctggaagtgtgacggagaagacgactgtggggacggctcagatgagcccaaggaagagtgtgatgagcgcacctgtgagccataccagttccgctgcaaaaacaaccgctgtgtgccaggccgctggcagtgtgactatgacaatgactgtggagataactcagacgaggagagctgcacacctcggccctgctctgagagtgaattttcctgtgccaacggccgctgcattgctgggcgctggaagtgtgacggcgatcatgactgtgccgacggctccgatgagaaagactgcaccccccgctgtgatatggaccagttccagtgcaagagtggtcactgcatccccctgcgctggcgctgtgatgcggatgctgactgtatggacggcagtgatgaggaagcctgcggcactggggtgaggacctgccccttggatgaatttcaatgtaacaacaccctgtgcaagccactggcctggaagtgtgacggagaggacgactgtggagacaactcagatgagaaccctgaggaatgcacccggttccagtgccctcctaaccgacccttccgctgcaagaatgaccgtgtctgcctgtggattgggcgccagtgtgacggcaccgacaactgtggggatgggactgacgaggaggactgtgagccccccacagcccagaacccccactgcaaagacaagaaggagttcctgtgccggaaccagcgctgtctgtcatcctcgctgcgctgtaacatgtttgatgactgtggcgatggctctgatgaagaagactgcagcatagaccccaagctgaccagctgtgccaccaatgccagcatgtgtggggacgaagcacgttgtgtgcgcaccgagaaggctgcctactgtgcctgccgcccgggcttccatactgtgccgggccagcccggatgccaggacatcaacgagtgcctgcgcttcggcacctgctctcagctctgcaacaataccaagggaggccacctctgcagctgtgcacgcaacttcatgaagacacacaatacctgcaaagctgaaggctccgagtaccaggtgctatacatcgctgatgacaacgagatccgaagcttgttcccggggcacccccactcagcctatgagcaggccttccagggtgacgagagtgtccgcatagatgccatggacgtccatgtcaaggccggccgtgtctactggactaactggcacacgggcactatctcctataggagcctaccccctgctgcccctcctaccacttccaaccgtcaccggaggcagatcgaccgtggagtcacccacctcaatatttcagggctgaagatgccgaggggcattgccatcgactgggtggctgggaatgtgtactggaccgactccggccgagacgtgattgaggtggcgcaaatgaagggagagaaccgcaagacgctcatctcgggcatgattgatgagccccacgccatcgtggtggacccactgaggggcaccatgtactggtcagactgggggaaccaccccaagattgaaacagccgcgatggatgggaccctacgggagaccctcgtgcaagacaacattcagtggcccacaggtctggccgtcgactatcacaatgaacggctgtactgggcggatgccaaactatcggtcatcggcagcatccggctcaacggcaccgaccccattgtggctgttgacagtaaacgaggcctgagtcaccccttcagcatcgacgtgttcgaggactacatctatggcgtcacttacatcaacaaccgtgtcttcaagatccacaagtttggacacagccccttgatcaacctgacagggggcctgagccacgcctctgatgtggtcctgtaccatcaacacaagcagcctgaagtgactaacccctgtgaccgcaagaaatgtgaatggctgtgtctgctgagccccagtgggcctgtctgcacctgtcccaatggaaagaggctggacaatggcacctgtgtgcctgtgccctctccgacaccccctccagatgcccctaggcctggaacctgtaccctgcagtgcttcaatggtggtagctgtttcctcaatgctcggaggcagcccaagtgccgctgccagccccgttacacaggcgataagtgtgagctggaccagtgctgggaatactgtcacaacggaggcacctgtgcagcctccccatctggcatgcccacgtgccgctgtcccacaggcttcacaggccccagatgcacccagcaggtgtgtgcaggctactgtgctaacaacagcacctgcaccgtcaaccagggtaaccagccccagtgccgatgtctacctggcttcctgggtgaccgttgccagtaccggcagtgctcaggcttctgtgagaactttggcacctgtcagatggccgccgatggctcccgacaatgtcgatgcactgtctactttgagggaacgaggtgtgaggtgaacaagtgtagtcgctgtctccagggagcctgtgtggtcaataagcagacgggagatgtcacctgcaactgcactgatggccgggtagctcccagttgtctgacctgcatcgaccactgtagcaatggtggctcctgcaccatgaacagcaagatgatgccagagtgccagtgcccaccccatatgacaggaccccggtgcgaggagcaggttgtcagtcagcaacagcctgggcatatgacctccatcctgatccctctgctgctgctgctcctgctgctgctggtggcaggcgtggtgttctggtataagcggcgagtccgaggggctaagggcttccagcaccagcggatgaccaatggggccatgaatgtggaaatcggaaaccctacctacaagatgtatgaaggtggagagcccgacgatgtggggggcctcctggatgctgattttgcccttgaccctgacaagcctaccaacttcaccaacccagtgtatgccacgctctacatggggggtcatggcagccgccactccctggccagcacggacgagaagcgagaactgctgggccggggacctgaagatgagataggggatcccttagcatagggccctgccccaacggacgtccccagaaagcccctgccacacgagtctttcaatgagccctctccccagccagcccttctccggccctgccggatgtacaaatgtaaaaatgaaggaattactttttatatgtgagtgagcaagcacagtattatctctttgcatttcctttctgcctgctcctcggcatcccctccccccatgctgccttgagggggcagggagggctctgtggctcaaaggtatgaaggagtccacatacgttcccttaccccgggaagctggcggcacagcctctcgcctgtacaagacactcaacagggctccagtgtcccagctttcctttcctggggttagttctggggaggtggagttctctgctgaacctgtctggaatatctggctctagctgaggtaggagtattttttagttgagggaagtcaccccaagccccagctcccacttttaggggcacgtctgggatggccatgctcagtatcccttccagacaggtctttgcctctccagtgccccctctgtggctcctagggctgaacacattctttggtaactgtcccccagtctcccctcccctgaggaccaggaagaattggggcacaccaaggaagggcaagtgggcagccccattttggggacgtgaacgttttaataatttttgctgaattcctttacaactaaataacacagatattgttataaataaaattgt

SEQ ID NO: 9 - protein, 5 aa, Artificial
  VHCDR1
SYAMS

SEQ ID NO: 10 - protein, 17 aa, Artificial
  VHCDR2
AISGSGGSTYYADSVKG

SEQ ID NO: 11 - protein, 8 aa, Artificial
  VHCDR3
RTGTLFDY

SEQ ID NO: 12 - protein, 11 aa, Artificial
  VLCDR1
QGDSLRSYYAS

SEQ ID NO: 13 - protein, 7 aa, Artificial
  VLCDR2
GKNNRPS

SEQ ID NO: 14 - protein, 11 aa, Artificial
  VLCDR3
NSSQAQRNAVV

SEQ ID NO: 15 - protein, 117 aa, Artificial
  VH
EVQLLESGGGLVQPGGSLRLSCAASGFTFSSYAMSWVRQAPGKGLEWVSAISGSGGSTYYADSVKGRFTISRDNSKNTLYLQMNSLRAEDTAVYYCAKRTGTLFDYWGQGTLVTVSS

SEQ ID NO: 16 - protein, 109 aa, Artificial
  VL
SSELTQDPAVSVALGQTVRITCQGDSLRSYYASWYQQKPGQAPVLVIYGKNNRPSGIPDRFSGSSSGNTASLTITGAQAEDEADYYCNSSQAQRNAVVFGGGTKLTVLG

SEQ ID NO: 17 - DNA, 351 bp, Artificial Sequence
  VH
gaagtccaactgctggaatcgggtggtggtctggtgcaaccgggcggctcgctgcgtctgtcatgtgctgcgtcgggctttacctttagctcttatgcaatgtcctgggtgcgtcaggcaccgggtaaaggtctggaatgggttagcgcaattagtggctccggcggtagcacctattacgccgattctgttaaaggtcgttttaccatctcacgcgacaactcgaaaaatacgctgtatctgcagatgaacagtctgcgcgcagaagataccgctgtctattactgcgcaaaacggactgggactttgttcgactactggggccaaggtacgctggttacggttagcagc

SEQ ID NO: 18 - DNA, 327 bp, Artificial Sequence
  VL
tcgtctgaactgacgcaagatccggctgtttctgtggcactgggtcaaacggttcgtatcacgtgtcaaggcgattcactgcgctcctattacgcaagttggtatcagcaaaaaccgggccaggctccggtgctggttatttacggcaaaaacaatcgtccgtccggtatcccggatcgcttttcaggcagctctagtggtaacaccgcgtcgctgaccattacgggtgcgcaagccgaagatgaagcagactattactgcaatagctcccaggcgcagcggaatgcggttgtctttggtggtggtacgaaactgaccgtcctgggc

SEQ ID NO: 19 - protein, 240 aa, Artificial Sequence
  scFv
EVQLLESGGGLVQPGGSLRLSCAASGFTFSSYAMSWVRQAPGKGLEWVSAISGSGGSTYYADSVKGRFTISRDNSKNTLYLQMNSLRAEDTAVYYCAKRTGTLFDYWGQGTLVTVSSGGGGSGGGGSGGGGSSELTQDPAVSVALGQTVRITCQGDSLRSYYASWYQQKPGQAPVLVIYGKNNRPSGIPDRFSGSSSGNTASLTITGAQAEDEADYYCNSSQAQRNAVVFGGGTKLTVLG

SEQ ID NO: 20 - DNA, 720 bp, Artificial Sequence
  scFv
gaagtccaactgctggaatcgggtggtggtctggtgcaaccgggcggctcgctgcgtctgtcatgtgctgcgtcgggctttacctttagctcttatgcaatgtcctgggtgcgtcaggcaccgggtaaaggtctggaatgggttagcgcaattagtggctccggcggtagcacctattacgccgattctgttaaaggtcgttttaccatctcacgcgacaactcgaaaaatacgctgtatctgcagatgaacagtctgcgcgcagaagataccgctgtctattactgcgcaaaacggactgggactttgttcgactactggggccaaggtacgctggttacggttagcagcggcggtggtggcagcggtggtggcggctcgggtggtggcggctcgtctgaactgacgcaagatccggctgtttctgtggcactgggtcaaacggttcgtatcacgtgtcaaggcgattcactgcgctcctattacgcaagttggtatcagcaaaaaccgggccaggctccggtgctggttatttacggcaaaaacaatcgtccgtccggtatcccggatcgcttttcaggcagctctagtggtaacaccgcgtcgctgaccattacgggtgcgcaagccgaagatgaagcagactattactgcaatagctcccaggcgcagcggaatgcggttgtctttggtggtggtacgaaactgaccgtcctgggc

SEQ ID NO: 21 - DNA, 29 bp, Artificial Sequence
  primer/ LRP1_C2_01
gcgatggatcctccggaggttccactagt

SEQ ID NO: 22 - DNA, 52 bp, Artificial Sequence
  primer/ LRP1_C2_06
gcatcaattgtcaggaaccagtagaagctccctcacagctcttctcatcgct

SEQ ID NO: 23 - DNA, 52 bp, Artificial Sequence
  primer/ LRP1_C2_08
gcatcaattgtcaggaaccagtagaagcggactcgcagttctcctcgtccga

SEQ ID NO: 24 - DNA, 52 bp, Artificial Sequence
  primer/ LRP1_C2_02
gcatcaattgtcaggaaccagtagaagcggctgaacaagtggcattggactc

SEQ ID NO: 25 - DNA, 52 bp, Artificial Sequence
  primer/ LRP1_C2_04
gcatcaattgtcaggaaccagtagaagcgttggtgcagttggcgtgtgtctc